European Patent Specification EP 3 833 780 B1, published August 27, 2025. Title: METHODS OF DETECTING INHERITED MYOPATHIES IN HORSES. Applicant: DIMMLER, KIRSTEN EDWARDS, JEREMY SCOTT SINCLAIR, ROBERT B. SZAUTER, PAUL. The sequence listing filed with the application follows.

SEQUENCE LISTING (264 sequences)

SEQ ID NO: 1 - DNA, 2001 bp, Equus caballus
ttcagttctaaatcatgataatttaaggaaaagtgccagctataaccactatgtttacccgaaagacaaaattctaatttattgttattattattattcccaaggcatgtttttattgtctttttcctccttagaaaattaatatatatttattgtagaaaacttggaaaatacagcacaatgaagagaataaaaatcactcacccaccttccgattgttattaacaaaataacattcttctattttagtatgctgttttttttaaaaagagttaatccataaagaaataactgttgattagaaattagaaccagtaaatatcttttttccatgaaacttgttttaatatttttaaatttcatctttttaaaaatattttgcctacatttaagaagcacagatatttacgaaacttcatttacttaaagttcaatggagaaaagtcttaatttatttctcagaatgtgagaaatccttacatcttataaagaataaagtggggtcatgtcgccacgtaagtttgacctctgagggaattgttagtaaagaatgttcgagccacttcaaaacgtcagcctccagggtccgaggtggggattgtgccaacggctgcatgaagtgaaccgggctgcatccttggcccagctctgggatctaacactggtggcttatttggggcagcctggcagctcttttgcagaactgtgggattttacagctgcaaggtaccttgatgggaaaatatgactgttcttacaatgctcctcctaattcttttttaatttccttcccaagaagccagcagggagggtggtccccgagatttctggctttctttgtggcgaggtcgggggaggtgggtgcctgactgttttccccttcctcctgctcatgccccttcctggctttcagatcagggtccaggtgatcgaggggcgccagctgccaggggtgaacatcaagcctgtggtcaaggtcaccgcggccaggcagaccaagyggactcggattcacaggggaaacagcccgctcttcaacgaggtgggagacatggcgttttagggctggtagcttggtgggccttccagattgggagcacccggcagatacctggcaattctttcagtttttgttcatggcgctaactttggtttgagaggtgtgccaggtcctgagtacgttatctgaggaactggagagagggttctagttcttattcctgtcccgggctcctggtgctccacatccctgtcttcctgtggggccagccacccatgctgtcctggagatgacaacctctgagaggtcaggggtggaacaccccagaacttgtcgagtcctcagagctcagggccgggcagagctcactctgtgctttccgtgtggaccagacctgaaggctgtgggtgtggccgaccctcttcccagcctgggggtcaacaggctctcgtttatcttcctttcgccctgaaccaacagactctcttcttcaacgtgtttgactctccctcggagctgtttgacgaggccgtctttatcacggtacgtctcagggatcaaggcgtgctctgtgggccgtgtgtacacacatgcattcagtgtgcatgtgtgtgtatgcacgtaggggtgtgagtgtgagagtgtgtaggagaagccttagggcccggggcctgggtgatgtggggagctcgctgctaagctctgctggtcacaaaagtgccttcagcagctcagatgaggcagcagcccagtggggagaccccccgctgctcagcacccccaggtgcctcaggccaggtcctgatatcattcctgcaggggatactttgattttcctctttttttctttgtccacttgcctgcttctggccaagattgcctctctctgagcctcagctctttgtttttcttccctctgaaaggcagtatagtttggtgaaaagcgtgggctttggagccaaactgtctggattctagtcctgcctgtgccatgtaggggc

SEQ ID NO: 2 - DNA, 1029 bp, Equus caballus
atacaggaggagaggaggacaccgaggaccaggggctcacgggagatgaggcagagccattcttggatcagaacggagccccaggccccggggctcccaccaccctgaagaagccaccttcccatcctcccccctaccatcctggggggaaaaggaagagaagcacgcctgcgcccagaaagctgctttcggataaaccacaggacttccagatcagggtccaggtgatcgaggggcgccagctgccaggggtgaacatcaagcctgtggtcaaggtcaccgcggccaggcagaccaagcggactcggattcacaggggaaacagcccgctcttcaacgagactctcttcttcaacgtgtttgactctccctcggagctgtttgacgaggccgtctttatcacggtggtagactcctgttcgctccggacagatgccctcatcggggagttccggatggatgtgggtaccatctacagagagccccgacacgcctatctcaggaagtggctgctgctctcggaccctgacgatttctctgctgggcccaaaggctacctgaaagcaagcctttgtgtgctggggcctggagacgaagctccgctggagagaaaggacccctctgaagacaaggaggacattgaaagcaatctgctcaggccaactggcatggcccttcgaggagcgcacttctgtctgaaggtcttcagggctgaggacttaccacagatggacgatgccgtggtggacagcgtgaagcagatcttcggctttgacagtaacaagaagaacctggtggatcccttcgtcgaggtcagctttgcggggaaaatgctctgcagcaagatcctggagaagatggccaaccctcagtggaaccagagcatcacgctgcctgtcatgtttccctccatgtctgaaaaaatgaggattcgtgtcatagactgggaccgcctcacccacaatgacatcgtggccaccacctacctgaatatgtcgaaaatctctgcccctggaggagaaatagcag

SEQ ID NO: 3 - DNA, 1029 bp, Artificial Sequence
  Description of Artificial Sequence: Synthetic polynucleotide
atacaggaggagaggaggacaccgaggaccaggggctcacgggagatgaggcagagccattcttggatcagaacggagccccaggccccggggctcccaccaccctgaagaagccaccttcccatcctcccccctaccatcctggggggaaaaggaagagaagcacgcctgcgcccagaaagctgctttcggataaaccacaggacttccagatcagggtccaggtgatcgaggggcgccagctgccaggggtgaacatcaagtctgtggtcaaggtcaccgcggccaggcagaccaagcggactcggattcacaggggaaacagcccgctcttcaacgagactctcttcttcaacgtgtttgactctccctcggagctgtttgacgaggccgtctttatcacggtggtagactcctgttcgctccggacagatgccctcatcggggagttccggatggatgtgggtaccatctacagagagccccgacacgcctatctcaggaagtggctgctgctctcggaccctgacgatttctctgctgggcccaaaggctacctgaaagcaagcctttgtgtgctggggcctggagacgaagctccgctggagagaaaggacccctctgaagacaaggaggacattgaaagcaatctgctcaggccaactggcatggcccttcgaggagcgcacttctgtctgaaggtcttcagggctgaggacttaccacagatggacgatgccgtggtggacagcgtgaagcagatcttcggctttgacagtaacaagaagaacctggtggatcccttcgtcgaggtcagctttgcggggaaaatgctctgcagcaagatcctggagaagatggccaaccctcagtggaaccagagcatcacgctgcctgtcatgtttccctccatgtctgaaaaaatgaggattcgtgtcatagactgggaccgcctcacccacaatgacatcgtggccaccacctacctgaatatgtcgaaaatctctgcccctggaggagaaatagcag

SEQ ID NO: 4 - DNA, 232 bp, Equus caballus
ctcctcccagatacaggaggagaggaggacaccgaggaccaggggctcacgggagatgaggcagagccattcttggatcagaacggagccccaggccccggggctcccaccaccctgaagaagccaccttcccatcctcccccctaccatcctggggggaaaaggaagagaagcacgcctgcgcccagaaagctgctttcggataaaccacaggacttccaggtgatgcacc

SEQ ID NO: 5 - DNA, 149 bp, Equus caballus
tggctttcagatcagggtccaggtgatcgaggggcgccagctgccaggggtgaacatcaagcctgtggtcaaggtcaccgcggccaggcagaccaagcggactcggattcacaggggaaacagcccgctcttcaacgaggtgggagaca

SEQ ID NO: 6 - DNA, 83 bp, Equus caballus
gaaccaacagactctcttcttcaacgtgtttgactctccctcggagctgtttgacgaggccgtctttatcacggtacgtctca

SEQ ID NO: 7 - DNA, 71 bp, Equus caballus
ttccctccaggtggtagactcctgttcgctccggacagatgccctcatcggggagttccgggtaattagtt

SEQ ID NO: 8 - DNA, 53 bp, Equus caballus
ctgattgcagatggatgtgggtaccatctacagagagccccgtgagtcatatt

SEQ ID NO: 9 - DNA, 136 bp, Equus caballus
tctctcttaggacacgcctatctcaggaagtggctgctgctctcggaccctgacgatttctctgctgggcccaaaggctacctgaaagcaagcctttgtgtgctggggcctggagacgaagctccggtgagtcatt

SEQ ID NO: 10 - protein, 342 aa, Equus caballus
TGGEEDTEDQGLTGDEAEPFLDQNGAPGPGAPTTLKKPPSHPPPYHPGGKRKRSTPAPRKLLSDKPQDFQIRVQVIEGRQLPGVNIKPVVKVTAARQTKRTRIHRGNSPLFNETLFFNVFDSPSELFDEAVFITVVDSCSLRTDALIGEFRMDVGTIYREPRHAYLRKWLLLSDPDDFSAGPKGYLKASLCVLGPGDEAPLERKDPSEDKEDIESNLLRPTGMALRGAHFCLKVFRAEDLPQMDDAVVDSVKQIFGFDSNKKNLVDPFVEVSFAGKMLCSKILEKMANPQWNQSITLPVMFPSMSEKMRIRVIDWDRLTHNDIVATTYLNMSKISAPGGEIA

SEQ ID NO: 11 - protein, 342 aa, Equus caballus
TGGEEDTEDQGLTGDEAEPFLDQNGAPGPGAPTTLKKPPSHPPPYHPGGKRKRSTPAPRKLLSDKPQDFQIRVQVIEGRQLPGVNIKPVVKVTAARQTKWTRIHRGNSPLFNETLFFNVFDSPSELFDEAVFITVVDSCSLRTDALIGEFRMDVGTIYREPRHAYLRKWLLLSDPDDFSAGPKGYLKASLCVLGPGDEAPLERKDPSEDKEDIESNLLRPTGMALRGAHFCLKVFRAEDLPQMDDAVVDSVKQIFGFDSNKKNLVDPFVEVSFAGKMLCSKILEKMANPQWNQSITLPVMFPSMSEKMRIRVIDWDRLTHNDIVATTYLNMSKISAPGGEIA

SEQ ID NO: 12 - DNA, 129 bp, Equus caballus
atcagggtccaggtgatcgaggggcgccagctgccaggggtgaacatcaagcctgtggtcaaggtcaccgcggccaggcagaccaagcggactcggattcacaggggaaacagcccgctcttcaacgag

SEQ ID NO: 13 - DNA, 129 bp, Artificial Sequence
  Description of Artificial Sequence: Synthetic polynucleotide
atcagggtccaggtgatcgaggggcgccagctgccaggggtgaacatcaagcctgtggtcaaggtcaccgcggccaggcagaccaagtggactcggattcacaggggaaacagcccgctcttcaacgag

SEQ ID NO: 14 - DNA, 20 bp, Artificial Sequence
  Description of Artificial Sequence: Synthetic primer
cccgagatttctggctttct

SEQ ID NO: 15 - DNA, 20 bp, Artificial Sequence
  Description of Artificial Sequence: Synthetic primer
ctcgacaagttctggggtgt

SEQ ID NO: 16 - DNA, 6243 bp, Homo sapiens
atgctgagggtcttcatcctctatgccgagaacgtccacacacccgacaccgacatcagcgatgcctactgctccgcggtgtttgcaggggtgaagaagagaaccaaagtcatcaagaacagcgtgaaccctgtatggaatgagggatttgaatgggacctcaagggcatccccctggaccagggctctgagcttcatgtggtggtcaaagaccatgagacgatggggaggaacaggttcctgggggaagccaaggtcccactccgagaggtcctcgccacccctagtctgtccgccagcttcaatgcccccctgctggacaccaagaagcagcccacaggggcctcgctggtcctgcaggtgtcctacacaccgctgcctggagctgtgcccctgttcccgccccctactcctctggagccctccccgactctgcctgacctggatgtagtggcagacacaggaggagaggaagacacagaggaccagggactcactggagatgaggcggagccattcctggatcaaagcggaggcccgggggctcccaccaccccaaggaaactaccttcacgtcctccgccccactaccccgggatcaaaagaaagcgaagtgcgcctacatctagaaagctgctgtcagacaaaccgcaggatttccagatcagggtccaggtgatcgaggggcgccagctgccgggggtgaacatcaagcctgtggtcaaggttaccgctgcagggcagaccaagcggacgcggatccacaagggaaacagcccactcttcaatgagactcttttcttcaacttgtttgactctcctggggagctgtttgatgagcccatctttatcacggtggtagactctcgttctctcaggacagatgctctcctcggggagttccggatggacgtgggcaccatttacagagagccccggcacgcctatctcaggaagtggctgctgctctcagaccctgatgacttctctgctggggccagaggctacctgaaaacaagcctttgtgtgctggggcctggggacgaagcgcctctggagagaaaagacccctctgaagacaaggaggacattgaaagcaacctgctccggcccacaggcgtagccctgcgaggagcccacttctgcctgaaggtcttccgggccgaggacttgccgcagatggacgatgccgtgatggacaacgtgaaacagatctttggcttcgagagtaacaagaagaacttggtggacccctttgtggaggtcagctttgcggggaaaatgctgtgcagcaagatcttggagaagacggccaaccctcagtggaaccagaacatcacactgcctgccatgtttccctccatgtgcgaaaaaatgaggattcgtatcatagactgggaccgcctgactcacaatgacatcgtggctaccacctacctgagtatgtcgaaaatctctgcccctggaggagaaatagaagaggagcctgcaggtgctgtcaagccttcgaaagcctcagacttggatgactacctgggcttcctccccacttttgggccctgctacatcaacctctatggcagtcccagagagttcacaggcttcccagacccctacacagagctcaacacaggcaagggggaaggtgtggcttatcgtggccggcttctgctctccctggagaccaagctggtggagcacagtgaacagaaggtggaggaccttcctgcggatgacatcctccgggtggagaagtaccttaggaggcgcaagtactccctgtttgcggccttctactcagccaccatgctgcaggatgtggatgatgccatccagtttgaggtcagcatcgggaactacgggaacaagttcgacatgacctgcctgccgctggcctccaccactcagtacagccgtgcagtctttgacgggtgccactactactacctaccctggggtaacgtgaaacctgtggtggtgctgtcatcctactgggaggacatcagccatagaatcgagactcagaaccagctgcttgggattgctgaccggctggaagctggcctggagcaggtccacctggccctgaaggcgcagtgctccacggaggacgtggactcgctggtggctcagctgacggatgagctcatcgcaggctgcagccagcctctgggtgacatccatgagacaccctctgccacccacctggaccagtacctgtaccagctgcgcacccatcacctgagccaaatcactgaggctgccctggccctgaagctcggccacagtgagctccctgcagctctggagcaggcggaggactggctcctgcgtctgcgtgccctggcagaggagccccagaacagcctgccggacatcgtcatctggatgctgcagggagacaagcgtgtggcataccagcgggtgcccgcccaccaagtcctcttctcccggcggggtgccaactactgtggcaagaattgtgggaagctacagacaatctttctgaaatatccgatggagaaggtgcctggcgcccggatgccagtgcagatacgggtcaagctgtggtttgggctctcagtggatgagaaggagttcaaccagtttgctgaggggaagctgtctgtctttgctgaaacctatgagaacgagactaagttggcccttgttgggaactggggcacaacgggcctcacctaccccaagttttctgacgtcacgggcaagatcaagctacccaaggacagcttccgcccctcggccggctggacctgggctggagattggttcgtgtgtccggagaagactctgctccatgacatggacgccggtcacctgagcttcgtggaagaggtgtttgagaaccagacccggcttcccggaggccagtggatctacatgagtgacaactacaccgatgtgaacggggagaaggtgcttcccaaggatgacattgagtgcccactgggctggaagtgggaagatgaggaatggtccacagacctcaaccgggctgtcgatgagcaaggctgggagtatagcatcaccatccccccggagcggaagccgaagcactgggtccctgctgagaagatgtactacacacaccgacggcggcgctgggtgcgcctgcgcaggagggatctcagccaaatggaagcactgaaaaggcacaggcaggcggaggcggagggcgagggctgggagtacgcctctctttttggctggaagttccacctcgagtaccgcaagacagatgccttccgccgccgccgctggcgccgtcgcatggagccactggagaagacggggcctgcagctgtgtttgcccttgagggggccctgggcggcgtgatggatgacaagagtgaagattccatgtccgtctccaccttgagcttcggtgtgaacagacccacgatttcctgcatattcgactatgggaaccgctaccatctacgctgctacatgtaccaggcccgggacctggctgcgatggacaaggactctttttctgatccctatgccatcgtctccttcctgcaccagagccagaagacggtggtggtgaagaacacccttaaccccacctgggaccagacgctcatcttctacgagatcgagatctttggcgagccggccacagttgctgagcaaccgcccagcattgtggtggagctgtacgaccatgacacttatggtgcagacgagtttatgggtcgctgcatctgtcaaccgagtctggaacggatgccacggctggcctggttcccactgacgaggggcagccagccgtcgggggagctgctggcctcttttgagctcatccagagagagaagccggccatccaccatattcctggttttgaggtgcaggagacatcaaggatcctggatgagtctgaggacacagacctgccctacccaccaccccagagggaggccaacatctacatggttcctcagaacatcaagccagcgctccagcgtaccgccatcgagatcctggcatggggcctgcggaacatgaagagttaccagctggccaacatctcctcccccagcctcgtggtagagtgtgggggccagacggtgcagtcctgtgtcatcaggaacctccggaagaaccccaactttgacatctgcaccctcttcatggaagtgatgctgcccagggaggagctctactgcccccccatcaccgtcaaggtcatcgataaccgccagtttggccgccggcctgtggtgggccagtgtaccatccgctccctggagagcttcctgtgtgacccctactcggcggagagtccatccccacagggtggcccagacgatgtgagcctactcagtcctggggaagacgtgctcatcgacattgatgacaaggagcccctcatccccatccaggaggaagagttcatcgattggtggagcaaattctttgcctccataggggagagggaaaagtgcggctcctacctggagaaggattttgacaccctgaaggtctatgacacacagctggagaatgtggaggcctttgagggcctgtctgacttttgtaacaccttcaagctgtaccggggcaagacgcaggaggagacagaagatccatctgtgattggtgaatttaagggcctcttcaaaatttatcccctcccagaagacccagccatccccatgcccccaagacagttccaccagctggccgcccagggaccccaggagtgcttggtccgtatctacattgtccgagcatttggcctgcagcccaaggaccccaatggaaagtgtgatccttacatcaagatctccatagggaagaaatcagtgagtgaccaggataactacatcccctgcacgctggagcccgtatttggaaagatgttcgagctgacctgcactctgcctctggagaaggacctaaagatcactctctatgactatgacctcctctccaaggacgaaaagatcggtgagacggtcgtcgacctggagaacaggctgctgtccaagtttggggctcgctgtggactcccacagacctactgtgtctctggaccgaaccagtggcgggaccagctccgcccctcccagctcctccacctcttctgccagcagcatagagtcaaggcacctgtgtaccggacagaccgtgtaatgtttcaggataaagaatattccattgaagagatagaggctggcaggatcccaaacccacacctgggcccagtggaggagcgtctggctctgcatgtgcttcagcagcagggcctggtcccggagcacgtggagtcacggcccctctacagccccctgcagccagacatcgagcaggggaagctgcagatgtgggtcgacctatttccgaaggccctggggcggcctggacctcccttcaacatcaccccacggagagccagaaggtttttcctgcgttgtattatctggaataccagagatgtgatcctggatgacctgagcctcacgggggagaagatgagcgacatttatgtgaaaggttggatgattggctttgaagaacacaagcaaaagacagacgtgcattatcgttccctgggaggtgaaggcaacttcaactggaggttcattttccccttcgactacctgccagctgagcaagtctgtaccattgccaagaaggatgccttctggaggctggacaagactgagagcaaaatcccagcacgagtggtgttccagatctgggacaatgacaagttctcctttgatgattttctgggctccctgcagctcgatctcaaccgcatgcccaagccagccaagacagccaagaagtgctccttggaccagctggatgatgctttccacccagaatggtttgtgtccctttttgagcagaaaacagtgaagggctggtggccctgtgtagcagaagagggtgagaagaaaatactggcgggcaagctggaaatgaccttggagattgtagcagagagtgagcatgaggagcggcctgctggccagggccgggatgagcccaacatgaaccctaagcttgaggacccaaggcgccccgacacctccttcctgtggtttacctccccatacaagaccatgaagttcatcctgtggcggcgtttccggtgggccatcatcctcttcatcatcctcttcatcctgctgctgttcctggccatcttcatctacgccttcccgaactatgctgccatgaagctggtgaagcccttcagctga

SEQ ID NO: 17 - protein, 2080 aa, Homo sapiens
MLRVFILYAENVHTPDTDISDAYCSAVFAGVKKRTKVIKNSVNPVWNEGFEWDLKGIPLDQGSELHVVVKDHETMGRNRFLGEAKVPLREVLATPSLSASFNAPLLDTKKQPTGASLVLQVSYTPLPGAVPLFPPPTPLEPSPTLPDLDVVADTGGEEDTEDQGLTGDEAEPFLDQSGGPGAPTTPRKLPSRPPPHYPGIKRKRSAPTSRKLLSDKPQDFQIRVQVIEGRQLPGVNIKPVVKVTAAGQTKRTRIHKGNSPLFNETLFFNLFDSPGELFDEPIFITVVDSRSLRTDALLGEFRMDVGTIYREPRHAYLRKWLLLSDPDDFSAGARGYLKTSLCVLGPGDEAPLERKDPSEDKEDIESNLLRPTGVALRGAHFCLKVFRAEDLPQMDDAVMDNVKQIFGFESNKKNLVDPFVEVSFAGKMLCSKILEKTANPQWNQNITLPAMFPSMCEKMRIRIIDWDRLTHNDIVATTYLSMSKISAPGGEIEEEPAGAVKPSKASDLDDYLGFLPTFGPCYINLYGSPREFTGFPDPYTELNTGKGEGVAYRGRLLLSLETKLVEHSEQKVEDLPADDILRVEKYLRRRKYSLFAAFYSATMLQDVDDAIQFEVSIGNYGNKFDMTCLPLASTTQYSRAVFDGCHYYYLPWGNVKPVVVLSSYWEDISHRIETQNQLLGIADRLEAGLEQVHLALKAQCSTEDVDSLVAQLTDELIAGCSQPLGDIHETPSATHLDQYLYQLRTHHLSQITEAALALKLGHSELPAALEQAEDWLLRLRALAEEPQNSLPDIVIWMLQGDKRVAYQRVPAHQVLFSRRGANYCGKNCGKLQTIFLKYPMEKVPGARMPVQIRVKLWFGLSVDEKEFNQFAEGKLSVFAETYENETKLALVGNWGTTGLTYPKFSDVTGKIKLPKDSFRPSAGWTWAGDWFVCPEKTLLHDMDAGHLSFVEEVFENQTRLPGGQWIYMSDNYTDVNGEKVLPKDDIECPLGWKWEDEEWSTDLNRAVDEQGWEYSITIPPERKPKHWVPAEKMYYTHRRRRWVRLRRRDLSQMEALKRHRQAEAEGEGWEYASLFGWKFHLEYRKTDAFRRRRWRRRMEPLEKTGPAAVFALEGALGGVMDDKSEDSMSVSTLSFGVNRPTISCIFDYGNRYHLRCYMYQARDLAAMDKDSFSDPYAIVSFLHQSQKTVVVKNTLNPTWDQTLIFYEIEIFGEPATVAEQPPSIVVELYDHDTYGADEFMGRCICQPSLERMPRLAWFPLTRGSQPSGELLASFELIQREKPAIHHIPGFEVQETSRILDESEDTDLPYPPPQREANIYMVPQNIKPALQRTAIEILAWGLRNMKSYQLANISSPSLVVECGGQTVQSCVIRNLRKNPNFDICTLFMEVMLPREELYCPPITVKVIDNRQFGRRPVVGQCTIRSLESFLCDPYSAESPSPQGGPDDVSLLSPGEDVLIDIDDKEPLIPIQEEEFIDWWSKFFASIGEREKCGSYLEKDFDTLKVYDTQLENVEAFEGLSDFCNTFKLYRGKTQEETEDPSVIGEFKGLFKIYPLPEDPAIPMPPRQFHQLAAQGPQECLVRIYIVRAFGLQPKDPNGKCDPYIKISIGKKSVSDQDNYIPCTLEPVFGKMFELTCTLPLEKDLKITLYDYDLLSKDEKIGETVVDLENRLLSKFGARCGLPQTYCVSGPNQWRDQLRPSQLLHLFCQQHRVKAPVYRTDRVMFQDKEYSIEEIEAGRIPNPHLGPVEERLALHVLQQQGLVPEHVESRPLYSPLQPDIEQGKLQMWVDLFPKALGRPGPPFNITPRRARRFFLRCIIWNTRDVILDDLSLTGEKMSDIYVKGWMIGFEEHKQKTDVHYRSLGGEGNFNWRFIFPFDYLPAEQVCTIAKKDAFWRLDKTESKIPARVVFQIWDNDKFSFDDFLGSLQLDLNRMPKPAKTAKKCSLDQLDDAFHPEWFVSLFEQKTVKGWWPCVAEEGEKKILAGKLEMTLEIVAESEHEERPAGQGRDEPNMNPKLEDPRRPDTSFLWFTSPYKTMKFILWRRFRWAIILFIILFILLLFLAIFIYAFPNYAAMKLVKPFS

SEQ ID NO: 18 - protein, 45 aa, Homo sapiens
FQIRVQVIEGRQLPGVNIKPVVKVTAAGQTKRTRIHKGNSPLFNE

SEQ ID NO: 19 - protein, 45 aa, Equus caballus
FQIRVQVIEGRQLPGVNIKPVVKVTAARQTKRTRIHRGNSPLFNE

SEQ ID NO: 20 - protein, 45 aa, Artificial Sequence
  Description of Artificial Sequence: Synthetic polypeptide
FQIRVQVIEGRQLPGVNIKPVVKVTAARQTKWTRIHRGNSPLFNE

SEQ ID NO: 21 - protein, 96 aa, Unknown
  Description of Unknown: DYSF sequence
PTSRKLLSDKPQDFQIRVQVIEGRQLPGVNIKPVVKVTAAGQTKRTRIHKGNSPLFNETLFFNLFDSPGELFDEPIFITVVDSRSLRTDALLGEFR

SEQ ID NO: 22 - protein, 96 aa, Unknown
  Description of Unknown: DYSF sequence
PTSRKLLSDKPQDFQIRVQVIEGRQLPGVNIKPVVKVTAAGQTKRTRIHKGNSPLFNETLFFNLFDCPAELFDEPIFITVVDSRSLRTDALLGEFR

SEQ ID NO: 23 - protein, 93 aa, Unknown
  Description of Unknown: DYSF sequence
RKLLSDKPQDFQIRVQVIEGRQLPGVNIKPVVKVTAAGQTKRTRIQKGNSPLFNETLFFNVFDSPLELFDEPIFITVVDSRSLRTDALLGEFR

SEQ ID NO: 24 - protein, 93 aa, Unknown
  Description of Unknown: DYSF sequence
RKLLSDKPQDFQIRVQVIEGRQLPGVNIKPVVKVTAAGQTKRTRIQKGNSPLFNETLFFNVFDSPSELFDEPIFITVVDSRSLRTDALLGEFR

SEQ ID NO: 25 - protein, 96 aa, Unknown
  Description of Unknown: DYSF sequence
PPPRKLLSDKPQDFQIRVQVIEGRQLPGVNIKPVVKVTAAGQTKRTRIHKGNSPLFNETLFFNLFDSPSELFDEPIFITVVDSRSLRTDALIGEFR

SEQ ID NO: 26 - protein, 96 aa, Unknown
  Description of Unknown: DYSF sequence
PAPRKVLSDKPQDFQIRVQVIEGRQLPGVNIKPVVKVTAAGQTRRTRIHKGNSPLFNETLFFNVFDSPAELFDEPIFITVVDSRSRRTDALIGEFR

SEQ ID NO: 27 - protein, 96 aa, Unknown
  Description of Unknown: DYSF sequence
PTPRKLLSDKPQDFQIRVQVIEGRQLPGVNIKPVVKVTAAGQTKRTRIHKGNSPLFNETLFFNVFDSPAELFDEPIFITVVDSRSLRTDALIGEFR

SEQ ID NO: 28 - protein, 96 aa, Unknown
  Description of Unknown: DYSF sequence
PAPRKLLSDKPQDFQIRVQVIEGRQLPGVNIKPVVKVTAARQTKRTRIHRGNSPLFNETLFFNVFDSPSELFDEAVFITVVDSCSLRTDALIGEFR

SEQ ID NO: 29 - protein, 96 aa, Unknown
  Description of Unknown: DYSF sequence
PTSRKLLSDKPQDFQIRVQVIEGRQLPGVNIKPVVKVTAAGQTKRTRIQKGNSPLFNETLFFNVFDSPSELFDEPIFITVVDSRSLRTDALIGEFR

SEQ ID NO: 30 - protein, 96 aa, Unknown
  Description of Unknown: DYSF sequence
PAPRKLLSDKPQDFQIRVQVIEGRQLPGVNIKPVVKVTAAGQTKRTRIHKGNSPFFNETLFFNVFDSPAELFNEPIFITVVDSRSLRTDALIGEFR

SEQ ID NO: 31 - protein, 96 aa, Cebus capucinus imitator
PTPRKLLSDKPQDFQIRVQVIEGRQLPGVNIKPVVKVTAAGQTKRTRIHKGNSPLFNETLFFNLFDSPAELFDEPIFITVVDSRSLRTDALLGEFR

SEQ ID NO: 32 - protein, 96 aa, Microcebus murinus
PPSRKLLSDKPQDFQIRVQVIEGRQLPGVNIKPVVKVTAAGQTKRTRIHKGNSPLFSETLFFNLFESPAELFDEPIFITVVDSRSLRTDALLGEFR

SEQ ID NO: 33 - protein, 96 aa, Carlito syrichta
PTSRKLLSDKPQDFQIRVQVIEGRQLPGVNIKPVVKVTAAGHTKRTRIQKGNNPLFSETLFFNLFDSPAELFDEPIFITVVDSRSLRTDALLGEFR

SEQ ID NO: 34 - protein, 93 aa, Otolemur garnettii
RKLLSDKPQDFQIRVQVIEGRQLPGVNIKPVVKVTAAGHTKRTRIHKGNSPLFNETLFFNLVESPAELFDEPIFITVVDSRSLRTDALLGEFR

SEQ ID NO: 35 - protein, 96 aa, Propithecus coquereli
PTSRKLLSDKPQDFQIRVQVIEGRQLPGVNIKPVVKVTAAGHTKRTRIQKGNNPLFNETLFFNLFDSPAELFDEPIFITVVDSRSLRTDALLGEFR

SEQ ID NO: 36 - protein, 93 aa, Cricetulus griseus
RKLLSDKPQDFQIRVQVIEGRQLPGVNIKPVVKVTAAGQTKRTRIQKGNSPVFNETLFFNVFDSPSELFDEPIFITVVDSRSLRTDALLGEFR

SEQ ID NO: 37 - protein, 96 aa, Ictidomys tridecemlineatus
PPSRKPLSDKQQDFQIRVQVIEGRQLPGVNIRPVVKVTAAGQTKRTRIHKGNSPFFNETLFFNVFDSPLELFDEPIFITVVDSCSLRTDALIGEFR

SEQ ID NO: 38 - protein, 96 aa, Marmota marmota marmota
PPSRKPLSDKQQDFQIRVQVIEGRQLPGVNIRPVVKVTAAGQTKRTRIHKGNSPLFNETLFFNVFDSPLELFDEPIFITVVDSCSLRTDALIGEFR

SEQ ID NO: 39 - protein, 96 aa, Castor canadensis
PTSRKLLSDKPQDFQIRVQVIEGRQLPGVNIRPVVKVTAAGQTKRTRIHKGNSPVFNETLFFNMFESPAELFDEPIFITVVDSRSLRTDALIGEFR

SEQ ID NO: 40 - protein, 96 aa, Mustela putorius furo
PTPRKLLSDKPQDFQIRVQVIEGRQLPGVNIKPVVKVTAAGQTKRTRIHKGNSPLFNETLFFNVFDSPSELFEEPIFITVVDSRSLRTDALIGEFR

SEQ ID NO: 41 - protein, 96 aa, Hipposideros armiger
PKARTLLSEKPQDFQIRVQVIEGRQLPGLNIKPVVKVTAAGQTKRTRIHKGNSPLFSETLFFNVFDSPAELFDEPIFITVVDSRSLRTDALIGEFR

SEQ ID NO: 42 - protein, 90 aa, Loxodonta africana
LSDKPQDFQIRVQVIEGRQLPGVNIKPVVKVTAAGQTKRTRIHKGNSPLFNETLFFNVCESPAQLFDEPIFITVVDSRSLRTDALIGEFR

SEQ ID NO: 43 - protein, 96 aa, Sus scrofa
PAPRKPLSDKPQDFQIRVQVIEGRQLPGVNIKPVVKVTAAGQTKRTRIHKGNSPLFNETLFFNVFDSPAELFNEPIFITVVDSRSLRTDALIGEFR

SEQ ID NO: 44 - protein, 96 aa, Bos taurus
PAPSKPLSDKPQDFQIRVQVIKGRQLPGVNIKPVVKVTAAGQTKRTRIHKGNSPVFNETLFFNVFDSPAELFNEPIFITVVDSRSLRTDALIGEFR

SEQ ID NO: 45 - protein, 96 aa, Balaenoptera acutorostrata scammoni
PAPRKLLSDKSQDFQIRVQVIEGRQLPGVNIKPVVKVTAAGQTKRTRIHKGNSPLFNETLFFNVFDSPAELFDEPIFITVVDSCSLRTDAFLGEFR

SEQ ID NO: 46 - protein, 96 aa, Ailuropoda melanoleuca
PTPRKLLSDKPQDFQIRVQVIEGRQLPGVNIKPVVKVTAAGQTKRTRIHKGNSPLFNETLFFNVFDSPSELFDEPIFITVVDSRSLRTDALIGEFR

SEQ ID NO: 47 - protein, 96 aa, Orcinus orca
PAPRKPLSDKSQDFQIRVQVIEGRQLPGVNIKPVVKVTAAGQTKRTRIHKGNSPLFNETLFFNVFDSPAELFDEPIFITVVDSCSLRTDALIGEFR

SEQ ID NO: 48 - protein, 95 aa, Phascolarctos cinereus
SSKKLLSDKPQDFQVRVQVIEGRQLPGLNIRPVVKVMACGQTKRTRIRKGNGPVFDETLFFNVFDSPVELFDEVICITVVDSRSLRTDALLGEFR

SEQ ID NO: 49 - protein, 89 aa, Sarcophilus harrisii
SDLSLCLQIRVQVVEGRQLPGVNIRPVVKVTAAGQTKRTRIRKGNSPVFDETLFFNVFDSPLELFDEPIFITVVDSRSLRTDALIGEFR

SEQ ID NO: 50 - protein, 78 aa, Ornithorhynchus anatinus
KIRVRVIEGRQLPGASIRPVVKVTAAGKTKRTRICKGNSPFFDETLFFNVFESPVELFEDPIFITVRTNASCRSPSPL

SEQ ID NO: 51 - protein, 85 aa, Homo sapiens
MLRVFILYAENVHTPDTDISDAYCSAVFAGVKKRTKVIKNSVNPVWNEGFEWDLKGIPLDQGSELHVVVKDHETMGRNRFLGEAK

SEQ ID NO: 52 - protein, 86 aa, Homo sapiens
MLCCLLVRASNLPSAKKDRRSDPVASLTFRGVKKRTKVIKNSVNPVWNEGFEWDLKGIPLDQGSELHVVVKDHETMGRNRFLGEAK

SEQ ID NO: 53 - protein, 96 aa, Homo sapiens; identical to SEQ ID NO: 21

SEQ ID NO: 54 - protein, 88 aa, Homo sapiens
ILAWGLRNMKSYQLANISSPSLVVECGGQTVQSCVIRNLRKNPNFDICTLFMEVMLPREELYCPPITVKVIDNRQFGRRPVVGQCTIR

SEQ ID NO: 55 - protein, 96 aa, Equus caballus; identical to SEQ ID NO: 28

SEQ ID NO: 56 - DNA, 2001 bp, Equus caballus
gactcttttttctccacgtcgggtctagggtgcagatgagtttatgggacgctgcatctgtcagccgactctggaacggatgccccggctgacctggttcccactgactaggggcagccagccggcgggcgagctgctggcctcttttgagctcatccagagagagaaggtgaggctggtccccatcctgatccaggaagcccagacagggagtacatggtaggagagggtagggggcacaggcagggatgccccgaaggaggggaggggctgccgatacatccttctccccccaccaggcctgctcagtggggagcactgaaccgccacctctggaattcaggcttcctgctgagactggttttgcccctcttttctgaaccccaagttaggctactgtctaaacattggggtagaatgttggaatctgggctgtgctggaatgtctgagtcctctggccattggatgtatttttccctgggtcatatcctgacgtggtttctgagaggaggacctccgtgatctggtcggggagacttaattgtgatggtggcacccagggacaggtaaggtcaggacctccggtgtagtgttggctctgccatggcctggctgtgcgaccctgggccaggcacttccctgctgtgaaatagggggtttgggttagaaccatatcttcagctttgctcttagagtgatgtgaaccccaggtgtaagctggatggaagtcaggctactctgggtcaagtgtctggagggggcacacagtatgctgcaacctggcttcccctggcacctggctgccaactcccgggcacctccaaggagtccctaggttgcaaactcccaactgtgatcactgacatattccatgagtgtcattttgtggctgaaggtgtgtttgcctggcccggacagaaaggagggtgatggggccttgggtgacaggcactgaccaaagctcttttttctaccccgcagccggccatctaccacattmctggttttgaggtaagtcttgctcttccctcttcttcttcaaactcatggcccgcctctgtgtgtttgcagccccctatgagctaggaagggcagtcaggtgtataccaccaccggcccgccttcagggatggggtgggtgagggccggggtccctggccagctcaggcctttcccgcccttcttccctgagactcagactgtagggacctcatggtcatccagcccacgggctctcagctgggctgcatgttagaatcccttcggcagcttgaaaaatcaccagtgctcaggccccaccccagaccagatggaacacagtctctggggatgtggcccaggcattggtatctttcagagcttcccaggggattttaatgtgctgctagggctgagcaccatcgacttagcccagtggttctcagtgtgatatcacctgggatgttgttagaaatgccgattcttggctcctgcttcacacctactgaagcaaactctgaggggcagtgcagcaacctgcaaattaacaagcctccaggggattctgatgcccactcgagtttcagaagctctggcttagaccatcttccccaactcattgttccccccatgaccggtttttcctcctctactagtgatgggggctctgttcccttctccctgctctccttccttctcctgggggcatggtagaaaatgcagaccctttcctggtacccaggctaatttgattcaggagatactgttctcagtcaggttcagctgcatcttggaggagcggtcatccggtctgtcgttggatgccttcccccttacaaggcagtccacgcaatctgcagacagtttttaccatgcaggccttccttcacccctgtctctgctccacccccggcatccctcagccccctctctctcctgctccctctcctgtccagcccaagctcccgctctcaggtctgccagcccctggggatccagattctttctccctggctctccaa

SEQ ID NO: 57 - DNA, 459 bp, Equus caballus
agacccacgatttcctgcatcttcgactacgggaaccgctaccatctacgctgctacatgtaccaggcccgggacctgcccgccatggacaaggactctttttctgatccctacgcaatcgtctccttcctgcaccagagccagaagacagtggtggtgaagaacaccctgaaccccacctgggaccagacactcatcttctatgagatcgagatctttggtgagccgcccagcatcgccgagcagccgcccagcatcgtggtggagctatacgaccatgacacctacggtgcagatgagtttatgggacgctgcatctgtcagccgactctggaacggatgccccggctgacctggttcccactgactaggggcagccagccggcgggcgagctgctggcctcttttgagctcatccagagagagaagccggccatctaccacattcctggttttgag

SEQ ID NO: 58 - DNA, 459 bp, Artificial Sequence
  Description of Artificial Sequence: Synthetic polynucleotide
agacccacgatttcctgcatcttcgactacgggaaccgctaccatctacgctgctacatgtaccaggcccgggacctgcccgccatggacaaggactctttttctgatccctacgcaatcgtctccttcctgcaccagagccagaagacagtggtggtgaagaacaccctgaaccccacctgggaccagacactcatcttctatgagatcgagatctttggtgagccgcccagcatcgccgagcagccgcccagcatcgtggtggagctatacgaccatgacacctacggtgcagatgagtttatgggacgctgcatctgtcagccgactctggaacggatgccccggctgacctggttcccactgactaggggcagccagccggcgggcgagctgctggcctcttttgagctcatccagagagagaagccggccatctaccacattactggttttgag

SEQ ID NO: 59 - DNA, 50 bp, Equus caballus
taccccgcagccggccatctaccacattcctggttttgaggtaagtcttg

SEQ ID NO: 60 - protein, 153 aa, Equus caballus
RPTISCIFDYGNRYHLRCYMYQARDLPAMDKDSFSDPYAIVSFLHQSQKTVVVKNTLNPTWDQTLIFYEIEIFGEPPSIAEQPPSIVVELYDHDTYGADEFMGRCICQPTLERMPRLTWFPLTRGSQPAGELLASFELIQREKPAIYHIPGFE

SEQ ID NO: 61 - protein, 153 aa, Artificial Sequence
  Description of Artificial Sequence: Synthetic polypeptide
RPTISCIFDYGNRYHLRCYMYQARDLPAMDKDSFSDPYAIVSFLHQSQKTVVVKNTLNPTWDQTLIFYEIEIFGEPPSIAEQPPSIVVELYDHDTYGADEFMGRCICQPTLERMPRLTWFPLTRGSQPAGELLASFELIQREKPAIYHITGFE

SEQ ID NO: 62 - DNA, 30 bp, Equus caballus
ccggccatctaccacattcctggttttgag

SEQ ID NO: 63 - DNA, 30 bp, Artificial Sequence
  Description of Artificial Sequence: Synthetic oligonucleotide
ccggccatctaccacattactggttttgag

SEQ ID NO: 64 - DNA, 20 bp, Artificial Sequence
  Description of Artificial Sequence: Synthetic primer
ggttgcaaactcccaactgt

SEQ ID NO: 65 - DNA, 20 bp, Artificial Sequence
  Description of Artificial Sequence: Synthetic primer
gatttttcaagctgccgaag

SEQ ID NO: 66 - protein, 60 aa, Homo sapiens
TRGSQPSGELLASFELIQREKPAIHHIPGFEVQETSRILDESEDTDLPYPPPQREANIYM

SEQ ID NO: 67 - protein, 60 aa, Equus caballus
TRGSQPAGELLASFELIQREKPAIYHIPGFEVQDTSGILEESEDTDLPYPPPQREANIYM

SEQ ID NO: 68 - protein, 60 aa, Artificial Sequence
  Description of Artificial Sequence: Synthetic polypeptide
TRGSQPAGELLASFELIQREKPAIYHITGFEVQDTSGILEESEDTDLPYPPPQREANIYM

SEQ ID NO: 69 - protein, 60 aa, Unknown; identical to SEQ ID NO: 66
  Description of Unknown: DYSF sequence

SEQ ID NO: 70 - protein, 59 aa, Unknown
  Description of Unknown: DYSF sequence
RGSQPSGELLASFELIQREKPAIHHIPGFEVQETSRILDESEDTDLPYPPPQREANIYM

SEQ ID NO: 71 - protein, 60 aa, Unknown
  Description of Unknown: DYSF sequence
TRGSQPAGELLAAFELIQREKPAIHHIPGFEMHETSRILDETEDTDLPYPPPQREANIYM

SEQ ID NO: 72 - protein, 60 aa, Unknown
  Description of Unknown: DYSF sequence
TRGSQPAGELLASFELIQREKPAIHHIPGFEVQDTSRILEESEDTDLPYPPPQREANIYM

SEQ ID NO: 73 - protein, 60 aa, Unknown
  Description of Unknown: DYSF sequence
TRGNQPAGELLASFELIQREKPAIHHIPGFEVQDTAGILEESEDTDLPYPPPQREANIYM

SEQ ID NO: 74 - protein, 59 aa, Unknown
  Description of Unknown: DYSF sequence
RGSQPAGELLASFELIQREKPAIHHIPGFEVQDTSGILEESEDTDLPYPPPQREANIYM

SEQ ID NO: 75 - protein, 60 aa, Unknown
  Description of Unknown: DYSF sequence
TRGSQPAGELLASFELIQREKPAIHHIPGFEVQDTTGILEESEDTDLPYPPPQREANIYM

SEQ ID NO: 76 - protein, 60 aa, Unknown
  Description of Unknown: DYSF sequence
TRGSQPAGELLASFELIQREKPAIHHIPGFEVQDTSGILEESEDTDLPYPPPQREANIYM

SEQ ID NO: 77 - protein, 60 aa, Papio anubis
TKGSQPTGELLASFELIQREKPAIHHIPGFEVQETSRILDESEDTDLPYPPPQREANIYM

SEQ ID NO: 78 - protein, 60 aa, Macaca mulatta
TRGSQPTGELLASFELIQREKPAIHHIPGFEVQETSRILDESEDTDLPYPPPQREANIYM

SEQ ID NO: 79 - protein, 60 aa, Rhinopithecus bieti
TRGSQPMGELLASFELIQREKPAIHHIPGFEVQETSRILDESEDTDLPYPPPQREANIYM

SEQ ID NO: 80 - protein, 59 aa, Microcebus murinus
RGSQPSGELLASFELIQREKPAIYHIPGFEVQDTSRILDESEDTDLPYPPPQREANVYM

SEQ ID NO: 81 - protein, 59 aa, Carlito syrichta
RGGQPSGELLAAFELIQREKPAIHHIPGFEVQDASRILDEAEDTDLPYPPPQREANVHM

SEQ ID NO: 82 - protein, 59 aa, Otolemur garnettii
RGSQPSGELLASFELIQREKPAIHHIPGFEVQDTARILDESEDTDLPYPPPQREANIYV

SEQ ID NO: 83 - protein, 59 aa, Propithecus coquereli
RGSQASGELLASFELIQREKPAIYHIPGFEVQDTSRILDESEDTDLPYPPPQREANVYM

SEQ ID NO: 84 - protein, 60 aa, Cricetulus griseus
TRGGQPAGELLAAFELIQREKPAIHHIPGFEMHETSRILDETEDTDLPYPPPQREANIYM

SEQ ID NO: 85 - protein, 60 aa, Microtus ochrogaster
TRGSQPAGELLAAFELIQREKPAIHHIPGFEMHETSSILEETEDTDLPYPPPQREANIYM

SEQ ID NO: 86 - protein, 60 aa, Meriones unguiculatus
TRGSQPAGELLAAFELIQREKPAIHHIPGFEVQETSRTLDETEDTDLPYPPPQREANIYM

SEQ ID NO: 87 - protein, 59 aa, Ictidomys tridecemlineatus
RGSQPAGELLASFELIQREKPAIYHIPGFEVQDTSRILDESEDTDLPYPPPQREANIYV

SEQ ID NO: 88 - protein, 60 aa, Chinchilla lanigera
TRGNQPAGELLASFELIQREKPAIHHIPGFEVQDTSRILDESEDTDLPYPPPQREANIYM

SEQ ID NO: 89 - protein, 59 aa, Marmota marmota marmota
RGSQPAGELLASFELIQREKPAIYHIPGFEVQDTSRILDESEDTDLPYPPPQREANVYV

SEQ ID NO: 90 - protein, 59 aa, Castor canadensis
RSSQPAGELLASFELIQREKPAIHHIPGFEVQDTSRILDESEDADLPYPPPQREVNIYM

SEQ ID NO: 91 - protein, 59 aa, Mustela putorius furo
RGSQPAGELLASFELIQREKPAIHHIPGFEVHDTSGILDESEDTDLPYPPPQREANIYM

SEQ ID NO: 92 - protein, 60 aa, Fukomys damarensis
TRGSQPAGELLASFELIQREKPAIHHIPGFEVQDTSRILDESEDTDLPYPPPQREANIYM

SEQ ID NO: 93 - protein, 60 aa, Myotis brandtii
TRGSQPAGELLASFELIQREKPAIHHIPGFEVQDASRILEESEDTDLPYPPPQREANIYM

SEQ ID NO: 94 - protein, 60 aa, Pteropus vampyrus
TRGSQPAGELLASFELIQREKPAIYHIPGFEVQDTSRILEESEDTDLPYPPPQREANIYI

SEQ ID NO: 95 - protein, 60 aa, Equus caballus; identical to SEQ ID NO: 67

SEQ ID NO: 96 - protein, 60 aa, Equus asinus
TRGSQLAGELLASFELIQREKPAIYHLPGFEVQDTSGILEESEDTDLPYPPPQREANIYM

SEQ ID NO: 97 - protein, 60 aa, Loxodonta africana
TRGSQAAGELLASFELIQREKPAIHHIPGFEVQDTSRILEESEDTDLPYPPPQREANIYM

SEQ ID NO: 98 - protein, 60 aa, Balaenoptera acutorostrata scammoni
TRGNQPAGELLASFELIQREKPAIHHIPGFEVQDTSGILEESEDTDLPYPPPQREANIYM

SEQ ID NO: 99 - protein, 60 aa, Ailuropoda melanoleuca
VRGSQPAGELLASFELIQREKPAIHHIPGFEVQDTSGILDESEDTDLPYPPPQREANIYM

SEQ ID NO: 100 - protein, 60 aa, Orcinus orca
TRGNQPAGELLASFELIQREKPAIYHIPGFEVQDTSGILEESEDTDLPYPPPQREANIYM

SEQ ID NO: 101 - protein, 60 aa, Phascolarctos cinereus
VRGSRPAGELLAAFELIMREKPATHHIPGFEPEEISGVADEIGDTDLPYPPPQREANIYV

SEQ ID NO: 102 - protein, 60 aa, Ornithorhynchus anatinus
TKKNKPAGDLLAAFELIQREKPSTHHSDPGFDPAVRTSRPLGKAGDSDLPYPPPQREPNV

SEQ ID NO: 103 - DNA, 2001 bp, Equus caballus
cttccagatttgctccctgttactgcatttctaaattttacttgagattcattctttccttgtgagggcaactatcagctatcatactcaagaatgaagcaagtgctttcccacatgtattatcttaatcctctactttgaggcaagtattttctcccttatttactgataagtagaaacacacacatacaaacacgtgcacaaggttcaaggagagtaaataatttgcccatgaaagatctaactcagttccttattaaatctttaaatcatgactccaggctaatgtagtctacatcctacatctacatatttgtatatgccttatattttttttttttttttgaggaagattgtgagctgacgtctattgccaatcttcctctttttgcttaaggaagacctgagctaacatctgtgccatcttcctgtattttgtatgtgggccactgccacagcattacttgatgaccggtgtgtaggtctgtgcctgggatccgaaccccaggccaccaaagcggagcgtgtgaacttaaccactacgccaccaggccggcccctccttagatatttttaatgttcatatagattatgtggtattatcatctgtaggataaatgtatgccattcaaatgttttctttggaactctctccagtgacacttttagctgtaaaattttgtgaacagattttctgctggccattctaaataacacaaaataactatatattgtgtttcctttttatactcactagaataacttctttatcgccttttatatataggttgtattgctgggaaaatacaatgcacagggcttaggttcagatcatgaattaatgctgagatgtaccaaaggacaagaatacgtcaaagtcgtcatgcaaaatgggcgaatgatgggagctgtcttaattggtgaaaccgatttagaagaaacatttgaaaacttgattttaaaccagatgaatctttcagcatacggagaagatctgctgsatccagatattgacatagaagattattttgactaaaaaggtcattccaagaaccacataaagttccaaataagacaaaaaagtcacacatcaataaagtaaatgattgcactgatttaatgatgaccacattgaagttaaaagtacagaagtgataatgatttcagtggaaaaatattaaaaaataaattctaaagataaaatcaattcaagtaacttatttacagatttttttcctaacacaaaattgaccaattatgtaagaattctcaagttattcatttctgtgttttaaacgtacacacattcatttgtgattttagctttggagcacatttagctaggctgttatctgctcagcccacaacttggtcttggttagtagaccagagccattctttgattggaaaacgtcaagaagcttgtaattttattttacttagagatgccgcaatatcttcttgctaatattatttgtattgataccttattccttttttgtttgaattctacagctattattttaacctgaaatcattcactttctgtcatgagcctgtgacttttcagtacaataacactaccatcaaaagagagttatgtgaaaagaaaaaatatagctaggtatatcacggcataaagagcttaagacagttatgtgaacttactcttttaaggagtttacataaaaaaagatttattttcccttgtttcatactgtaaatttatacaattcatgctctcaaattttcaaaagatctcaaattctcaagtcctcaattctttagagataagttcttaaaatatagctccatttgtataaaacattaatgaaattgtcttaaaaattaaactttgattaactacaaaaataatggtgtaaacatgcataaactgttctgttcttggaaaatttagatacactcatgcatcatcaatttttcttttcttagcccctgtgttcttagcctcagattgctgaagcatgtttgcagacttct

SEQ ID NO: 104 - DNA, 1346 bp, Equus caballus
aggtttccagagtattggaagaatttgatgttgaagaacagccaaataccatgttagaaaatcgctttcccaacattaaggttatagaatctggagtaaagcaactgaagagtgaagaacactgcattttaacagaagatggcaatcagcatgtatataagaaactctgtctgtgtgctggagctaaaccaaagttgatatgtgaaggaaatccttatgtattaggaatccgtgacacagacagtgctcaggaatttcagaaacagcttactaaggctaaaagaataatgatcataggcaatggtgggatcgcacttgaattagtgtatgaaattgaaggctgtgaagtcatttgggtcattaaagacaaagctattgggaatacgttcttcgatgcaggagcagctgaattcttgacttcaaagctcatcgctgaaaaaccagagggtaaaattgcacatagaagaaccagatatacaactgaaggaaggaaaaaggaagcacgaaccaaaggtgatgctgctaatgtaggcagtgccctgggacctgactggcatgaaggcttgaatcttaaaggaacaaaagagttttctcataagattcacattgaaactatgtgtgaagtaaagaaaatctaccttcaggaagaatttagaatttccaagaaaaagtccttgacttttccaagagaccataataatcagtcagtttcaactgataaagagatatggcctgtatatgtggaattgaccaatgaaaagatatatggctgcgatttcattgtcagtgctacaggagttacaccaaatatagaacctttcctctgtggcaacaattttgatctaggagaagatggtggcctgaaagtgaataatcatatgcacacgtcccttcctgacatctatgctgcaggtgacatctgcactgcctcctgggaacccagcccagtgtggcagcagatgaggctgtggacgcaggctagacagatgggatggtatgcagccaagtgcatggctgcagctactttaggagactccattgacatggatttcagcttcgaactgtttgctcatgtaacaaaattttttaactataaggttgtattgctgggaaaatacaatgcacagggcttaggttcagatcatgaattaatgctgagatgtaccaaaggacaagaatacgtcaaagtcgtcatgcaaaatgggcgaatgatgggagctgtcttaattggtgaaaccgatttagaagaaacatttgaaaacttgattttaaaccagatgaatctttcagcatatggagaagatctgctggatccagatattgacatagaagattattttgactaa

SEQ ID NO: 105 - DNA, 1346 bp, Artificial Sequence
  Description of Artificial Sequence: Synthetic polynucleotide
aggtttccagagtattggaagaatttgatgttgaagaacagccaaataccatgttagaaaatcgctttcccaacattaaggttatagaatctggagtaaagcaactgaagagtgaagaacactgcattttaacagaagatggcaatcagcatgtatataagaaactctgtctgtgtgctggagctaaaccaaagttgatatgtgaaggaaatccttatgtattaggaatccgtgacacagacagtgctcaggaatttcagaaacagcttactaaggctaaaagaataatgatcataggcaatggtgggatcgcacttgaattagtgtatgaaattgaaggctgtgaagtcatttgggtcattaaagacaaagctattgggaatacgttcttcgatgcaggagcagctgaattcttgacttcaaagctcatcgctgaaaaaccagagggtaaaattgcacatagaagaaccagatatacaactgaaggaaggaaaaaggaagcacgaaccaaaggtgatgctgctaatgtaggcagtgccctgggacctgactggcatgaaggcttgaatcttaaaggaacaaaagagttttctcataagattcacattgaaactatgtgtgaagtaaagaaaatctaccttcaggaagaatttagaatttccaagaaaaagtccttgacttttccaagagaccataataatcagtcagtttcaactgataaagagatatggcctgtatatgtggaattgaccaatgaaaagatatatggctgcgatttcattgtcagtgctacaggagttacaccaaatatagaacctttcctctgtggcaacaattttgatctaggagaagatggtggcctgaaagtgaataatcatatgcacacgtcccttcctgacatctatgctgcaggtgacatctgcactgcctcctgggaacccagcccagtgtggcagcagatgaggctgtggacgcaggctagacagatgggatggtatgcagccaagtgcatggctgcagctactttaggagactccattgacatggatttcagcttcgaactgtttgctcatgtaacaaaattttttaactataaggttgtattgctgggaaaatacaatgcacagggcttaggttcagatcatgaattaatgctgagatgtaccaaaggacaagaatacgtcaaagtcgtcatgcaaaatgggcgaatgatgggagctgtcttaattggtgaaaccgatttagaagaaacatttgaaaacttgattttaaaccagatgaatctttcagcatatggagaagatctgctgcatccagatattgacatagaagattattttgactaa

SEQ ID NO: 106 - DNA, 269 bp, Equus caballus
ttatatataggttgtattgctgggaaaatacaatgcacagggcttaggttcagatcatgaattaatgctgagatgtaccaaaggacaagaatacgtcaaagtcgtcatgcaaaatgggcgaatgatgggagctgtcttaattggtgaaaccgatttagaagaaacatttgaaaacttgattttaaaccagatgaatctttcagcatacggagaagatctgctggatccagatattgacatagaagattattttgactaaaaaggtcatt

SEQ ID NO: 107 - protein, 447 aa, Equus caballus
VSRVLEEFDVEEQPNTMLENRFPNIKVIESGVKQLKSEEHCILTEDGNQHVYKKLCLCAGAKPKLICEGNPYVLGIRDTDSAQEFQKQLTKAKRIMIIGNGGIALELVYEIEGCEVIWVIKDKAIGNTFFDAGAAEFLTSKLIAEKPEGKIAHRRTRYTTEGRKKEARTKGDAANVGSALGPDWHEGLNLKGTKEFSHKIHIETMCEVKKIYLQEEFRISKKKSLTFPRDHNNQSVSTDKEIWPVYVELTNEKIYGCDFIVSATGVTPNIEPFLCGNNFDLGEDGGLKVNNHMHTSLPDIYAAGDICTASWEPSPVWQQMRLWTQARQMGWYAAKCMAAATLGDSIDMDFSFELFAHVTKFFNYKVVLLGKYNAQGLGSDHELMLRCTKGQEYVKVVMQNGRMMGAVLIGETDLEETFENLILNQMNLSAYGEDLLDPDIDIEDYFD

SEQ ID NO: 108 - protein, 447 aa, Equus caballus
VSRVLEEFDVEEQPNTMLENRFPNIKVIESGVKQLKSEEHCILTEDGNQHVYKKLCLCAGAKPKLICEGNPYVLGIRDTDSAQEFQKQLTKAKRIMIIGNGGIALELVYEIEGCEVIWVIKDKAIGNTFFDAGAAEFLTSKLIAEKPEGKIAHRRTRYTTEGRKKEARTKGDAANVGSALGPDWHEGLNLKGTKEFSHKIHIETMCEVKKIYLQEEFRISKKKSLTFPRDHNNQSVSTDKEIWPVYVELTNEKIYGCDFIVSATGVTPNIEPFLCGNNFDLGEDGGLKVNNHMHTSLPDIYAAGDICTASWEPSPVWQQMRLWTQARQMGWYAAKCMAAATLGDSIDMDFSFELFAHVTKFFNYKVVLLGKYNAQGLGSDHELMLRCTKGQEYVKVVMQNGRMMGAVLIGETDLEETFENLILNQMNLSAYGEDLLHPDIDIEDYFD

SEQ ID NO: 109 - DNA, 249 bp, Equus caballus
gttgtattgctgggaaaatacaatgcacagggcttaggttcagatcatgaattaatgctgagatgtaccaaaggacaagaatacgtcaaagtcgtcatgcaaaatgggcgaatgatgggagctgtcttaattggtgaaaccgatttagaagaaacatttgaaaacttgattttaaaccagatgaatctttcagcatatggagaagatctgctggatccagatattgacatagaagattattttgactaa

SEQ ID NO: 110 - DNA, 249 bp, Artificial Sequence
  Description of Artificial Sequence: Synthetic polynucleotide
gttgtattgctgggaaaatacaatgcacagggcttaggttcagatcatgaattaatgctgagatgtaccaaaggacaagaatacgtcaaagtcgtcatgcaaaatgggcgaatgatgggagctgtcttaattggtgaaaccgatttagaagaaacatttgaaaacttgattttaaaccagatgaatctttcagcatatggagaagatctgctgcatccagatattgacatagaagattattttgactaa

SEQ ID NO: 111 - DNA, 20 bp, Artificial Sequence
  Description of Artificial Sequence: Synthetic primer
cagattttctgctggccatt

SEQ ID NO: 112 - DNA, 23 bp, Artificial Sequence
  Description of Artificial Sequence: Synthetic primer
tggtcatcattaaatcagtgcaa

SEQ ID NO: 113 - DNA, 1012 bp, Homo sapiens
tgaaattgaaggctgtgaagtgatttgggccattaaagataaagctatagggaatactttcttcgatgcaggagcagctgaattcttgacttcaaagctcattgctgaaaaatcagaggctaaaattgcacataaaagaaccagatatacaactgaaggaaggaaaaaggaagctagaagcaaatctaaagcagataatgtaggaagtgcattgggaccagattggcatgaaggcttgaatcttaaaggaacaaaagagttttctcataagattcaccttgaaactatgtgtgaagtaaagaaaatctaccttcaggatgagtttagaattttgaagaaaaagtccttcacttttccaagagaccataagtcagttacagctgatacagagatgtggcctgtctatgtggaattgaccaatgaaaagatatatggctgcgatttcattgtcagtgctacaggagttacaccaaatgtagaaccttttctccatggtaacagttttgatctaggagaagatggtggcctgaaagtggatgatcatatgcacacatcccttcctgatatctatgctgccggtgacatctgtactacatcctggcagctgagcccagtctggcagcagatgaggctgtggacccaggctagacagatgggatggtatgcagcaaagtgcatggctgcagcgagttcaggagactctattgacatggatttcagctttgaactgtttgctcatgtgacaaaattttttaactataaggttgtactgctgggaaaatacaatgcacagggcttaggttcagatcatgaattaatgctgagatgtaccaaaggacgagaatacatcaaagtcgtcatgcaaaatggacgaatgatgggagctgtcttaattggtgaaaccgatttagaagaaacatttgaaaacctaatcttaaaccaaatgaatctttcatcatatggagaagatctgctagatccaaatattgatatagaagattattttgactaa

SEQ ID NO: 114 - protein, 445 aa, Homo sapiens
ISKILEEFDVEEQSSTMLGKRFPNIKVIESGVKQLKSEEHCIVTEDGNQHVYKKLCLCAGAKPKLICEGNPYVLGIRDTDSAQEFQKQLTKAKRIMIIGNGGIALELVYEIEGCEVIWAIKDKAIGNTFFDAGAAEFLTSKLIAEKSEAKIAHKRTRYTTEGRKKEARSKSKADNVGSALGPDWHEGLNLKGTKEFSHKIHLETMCEVKKIYLQDEFRILKKKSFTFPRDHKSVTADTEMWPVYVELTNEKIYGCDFIVSATGVTPNVEPFLHGNSFDLGEDGGLKVDDHMHTSLPDIYAAGDICTTSWQLSPVWQQMRLWTQARQMGWYAAKCMAAASSGDSIDMDFSFELFAHVTKFFNYKVVLLGKYNAQGLGSDHELMLRCTKGREYIKVVMQNGRMMGAVLIGETDLEETFENLILNQMNLSSYGEDLLDPNIDIEDYFD

SEQ ID NO: 115 - protein, 82 aa, Homo sapiens
VVLLGKYNAQGLGSDHELMLRCTKGREYIKVVMQNGRMMGAVLIGETDLEETFENLILNQMNLSSYGEDLLDPNIDIEDYFD

SEQ ID NO: 116 - protein, 82 aa, Equus caballus
VVLLGKYNAQGLGSDHELMLRCTKGQEYVKVVMQNGRMMGAVLIGETDLEETFENLILNQMNLSAYGEDLLDPDIDIEDYFD

SEQ ID NO: 117 - protein, 82 aa, Artificial Sequence
  Description of Artificial Sequence: Synthetic polypeptide
VVLLGKYNAQGLGSDHELMLRCTKGQEYVKVVMQNGRMMGAVLIGETDLEETFENLILNQMNLSAYGEDLLHPDIDIEDYFD

SEQ ID NO: 118 - protein, 60 aa, Unknown
  Description of Unknown: PYROXD1 sequence
TKGQEYIKVVMQNGRMMGAVLIGETDLEETFENLILNQMNLSSYGEDLLDPNIDIEDYFD

SEQ ID NO: 119 - protein, 60 aa, Unknown
  Description of Unknown: PYROXD1 sequence
TKGQEYVKVVMQNGRMMGAVLIGETDLEETFENLILNQMNLSSYGEDLLDPNIDIEDYFD

SEQ ID NO: 120 - protein, 60 aa, Unknown
  Description of Unknown: PYROXD1 sequence
TRGQEYVKVVMQNGRMMGAVLIGETDLEETFENLILNQMDLSSYGEDLLDPNIDIEDYFD

SEQ ID NO: 121 - protein, 60 aa, Unknown
  Description of Unknown: PYROXD1 sequence
TKGQEYVKVVMQNGRMMGAVLIGETDLEETFENLILNQMDLSSYGEDLLDPNIDIEDYFD

SEQ ID NO: 122 - protein, 60 aa, Unknown
  Description of Unknown: PYROXD1 sequence
TKGQEYIKVVMQNGRMMGAVLIGETNLEETFENLILNQMNLSSYGEDLLDPNIDIEDYFD

SEQ ID NO: 123 - protein, 60 aa, Unknown
  Description of Unknown: PYROXD1 sequence
TKGQEYVKVVMQNGRMMGAVLIGETDLEETFENLILNQMNLSAYGEDLLDPDIDIEDYFD

SEQ ID NO: 124 - protein, 60 aa, Unknown
  Description of Unknown: PYROXD1 sequence
TKGQEYIKAVLQNGRMMGAVLIGETDLEETFENLILNQMNLSAYGEDLLDPNIDIEDYFD

SEQ ID NO: 125 - protein, 60 aa, Unknown
  Description of Unknown: PYROXD1 sequence
TKGQEYVKVVMQNGRMMGAVLIGETDLEETFENLILNQMDLSSYGEDLLDPNIDLEDYFD

SEQ ID NO: 126 - protein, 60 aa, Homo sapiens
TKGREYIKVVMQNGRMMGAVLIGETDLEETFENLILNQMNLSSYGEDLLDPNIDIEDYFD

SEQ ID NO: 127 - protein, 60 aa, Otolemur garnettii
TKGQEYIKVVMQNGRMMGAVLIGETDLEETFENLILNQMNLSQYGEDLLDPNIDIEDYFD

SEQ ID NO: 128 - protein, 60 aa, Rattus norvegicus
TRGQEYIKVVMHNGRMMGAVLIGETDLEETFENLILNQMDLSSYGEDLLNPDIDIEDYFD

SEQ ID NO: 129 - protein, 60 aa, Cricetulus griseus
TRGQEYIKVVMQNGRMMGAVLIGETDLEETFENLILNQMDLSSYGEDLLDPNIDIEDYFD

SEQ ID NO: 130 - protein, 60 aa, Microtus ochrogaster
TRGQEYVKVVMQNGRMMGAVLIGETDLEETFENLILNQMDLSSYGEDLLDPDIDIEDYFD

SEQ ID NO: 131 - protein, 60 aa, Chinchilla lanigera
TKGQEYVKVVMQNGRMMGAVLIGETDLEETFENLILNQMDLSPYGEELLDPNIDIEDYFD

SEQ ID NO: 132 - protein, 60 aa, Castor canadensis
TKGQEYIKVIMQNGRMMGAVLIGETDLEETFENLILNQMDLSSYGEDLLDPNIDIEDYFD

SEQ ID NO: 133 - protein, 60 aa, Mustela putorius furo
TKGQEYVKVVMQHGRMMGAVLIGETDLEETFENLILNQTDLSSYGEDLLDPNIDLEDYFD

SEQ ID NO: 134 - protein, 60 aa, Fukomys damarensis
TKGQEYIKVVMQNGHMMGAVLIGETDLEETFENLILNQMDLSPYGEDLLDPNIDIEDYFD

SEQ ID NO: 135 - protein, 60 aa, Vicugna pacos
TKGQEYVKAVLQNGRMMGAVLIGETDLEETFENLILNQMNLSAYGEDLLDPNIDIEDYFD

SEQ ID NO: 136 - protein, 60 aa, Ailuropoda melanoleuca
TKGQEYVKVVMQNGRMMGAVLIGETDLEETFENLILNQTDLSSYGEDLLDPNIDLEDYFD

SEQ ID NO: 137 - protein, 60 aa, Phascolarctos cinereus
TKGQEYVKVVMQNGRMMGAILIGETDLEETFENLILNQMNLSAYGEDLLDPDIDIEDYFD

SEQ ID NO: 138 - protein, 60 aa, Sarcophilus harrisii
TKGQEYVKVVMQNGRMMGAILIGETDLEETFENLILNQMNLSAYGEDLLDPNIDIEDYFD

SEQ ID NO: 139 - protein, 60 aa, Monodelphis domestica
TKGQEYVKVVMQNGRMMGAILIGETNLEETFENLILNQMNLSAYGEDLLDPSIDIEDYFD

SEQ ID NO: 140 - protein, 60 aa, Unknown
  Description of Unknown: PYROXD1 sequence
TKGQEYVKVVMQNGRMMGAVLIGETDLEETFENLILNQMDLSAYGEDLLNPDIDIEDYFD

SEQ ID NO: 141 - protein, 60 aa, Unknown
  Description of Unknown: PYROXD1 sequence
TKGHEYVKVVMQNGRMMGAVLIGETDLEETFENLILNQMDLSAYGEDLLNPDIDIEDYFD

SEQ ID NO: 142 - protein, 60 aa, Merops nubicus
TKGQEYVKVVMQNGRMVGAVLIGETDLEETFENLILNQMDLSAYGEDLLNPDIDIEDYFD

SEQ ID NO: 143 - protein, 60 aa, Apteryx australis mantelli
TKGQEYVKVVMQNGRMMGAVLIGETDLEETFENLILNQMDLSAYGEDLLNPNIDIEDYFD

SEQ ID NO: 144 - protein, 60 aa, Corvus brachyrhynchos
TKGHEYVKVVMQNGRMMGAVLIGETDLEETFENLILNRMDLSAYGEDLLNPDIDIEDYFD

SEQ ID NO: 145 - protein, 60 aa, Corvus cornix cornix; identical to SEQ ID NO: 144

SEQ ID NO: 146 - protein, 60 aa, Serinus canaria
TKGHEYIKVVMQNGRMMGAVLIGETDLEETFENLILNQMDLSAYGEDLLNPDIDIEDYFD

SEQ ID NO: 147 - protein, 60 aa, Sturnus vulgaris
TKGHEYVKVVMQNGRMMGAVLIGETDLEETFENLILNQIDLSAYGEDLLNPDIDLEDYFD

SEQ ID NO: 148 - protein, 60 aa, Lepidothrix coronata
TKGQEYVKAVMQNGRMVGAVLIGETDLEETFENLILNQMDLSAYGEDLLNPDIDIEDYFD

SEQ ID NO: 149 - protein, 60 aa, Amazona aestiva
TKGQEYVKVVMQSGRMVGAVLIGDTDLEETFENLILNQMDLSAYGEDLLNPDVDIEDYFD

SEQ ID NO: 150 - protein, 60 aa, Gekko japonicus
TKGQEYVKVVMQNGRMMGAVLIGETDLEETFENLILNQMDLSRYGEDLLDPNIDIEDYFD

SEQ ID NO: 151 - protein, 60 aa, Anolis carolinensis
TKGLEYVKVVMQNGRMLGAVLIGETDLEETFENLILNQMDLSRYGEDLLDPNIDIEDYFD

SEQ ID NO: 152 - protein, 60 aa, Python bivittatus
TKGQEYVKVVMQNGRMLGAVLIGETDLEETFENLILNQMDLSRYGEDLLDPNIDIEDYFD

SEQ ID NO: 153 - protein, 60 aa, Pogona vitticeps
TKGQEYIKVVMQNGRMLGAVLIGETDLEETFENLILNQMDLSRYGENLLDPNIDIEDYFD

SEQ ID NO: 154 - protein, 60 aa, Protobothrops mucrosquamatus
TKGQEYIKVVMQNGRMLGAVLIGETDLEETFENLILNQMDLSRYGEDLLDPNIDIEDYFD

SEQ ID NO: 155 - protein, 60 aa, Ophiophagus hannah
TKGQEYIKVVMQHGRMLGAVLIGETDLEETFENLILNQMDLSRYGEDLLDPNIDIEDYFD

SEQ ID NO: 156 - protein, 60 aa, Thamnophis sirtalis
TKGQEYIKVVMQNGRMLGAVLIGETDLEETFENLILNQMDLSRYGKDLLDPNIDIEDYFD

SEQ ID NO: 157 - protein, 60 aa, Latimeria chalumnae
TKGQEYVKVVLQNGRMMGAILIGETDLEETFENLMLNQMDLSAYGEELLNPDIDIEDYFD

SEQ ID NO: 158 - protein, 60 aa, Rhincodon typus
TTGQEYVKTVMQNGRMKGAVLIGETDLEETFENLILNQMDLSAYGEDLLNPNIDIEDYFD

SEQ ID NO: 159 - protein, 60 aa, Callorhinchus milii
TKGHEYVKAVMQNGRMMGAVLIGETNLEETFENLILNQMDLSSYGEELLNPNIDIEDYFD

SEQ ID NO: 160 - protein, 60 aa, Salmo salar
TKGHEYVKVVLSGGRMLGAVLIGETDLEETFENLILNQMDLTPYGEELLNPNIDIEDYFD

SEQ ID NO: 161 - protein, 60 aa, Xenopus laevis
TRGHEYVKLVMQGGRMVGALLIGDTDLEETFENLILNQTDLSSYGERLLDPNIDIEDYFD

SEQ ID NO: 162 - protein, 60 aa, Cyprinus carpio
TKGQEYVKVVLTGGRMVGAVLIGETDLEETFENLILNQMDLSRYGEELLNPNIDIEDYFD

SEQ ID NO: 163 - DNA, 2001 bp, Equus caballus
ttagaattctggggtggctggaggtgtgtttgctctctagctgcaaagataaacgtttgcaagacctgtcatacgaagacctgagaagtttccctaaaatgtggtctcagggtactttaagtttgttttaagaaaagagaagagttcgtagcttttcttgtttcaggctctataaaacctgtaagtttttgtaggtgaccattgcggggaccggcctcttcttgtccatgaggccagagtagcctggggcatcgtgcttcctggggaggaagaagcattgcccccctgttggggcagagagtgggtgctgaccgcatggtcagggtctgtcagaggcaggtggacgttctgtggatgggatgtgactgaagggacccgtctcttgagcctcacattcatatcatcacgaatatttttctgagcacctgatcctgcggcggtggctttcctcgcacatgtggctcatttccctgacttgtgttgttttcagggtgactcagggcgggacagccagcagagaggacccaaaggagaaaccggagacctcgggcccatggtacgatgctccttgttcccagactctcctgtgctggaggccagagaaacaaagctcacactggctcgccaggggccgaaggaccatggaagtggtctttgaggctggggagcatatgcggtcaggaacagagggccccgtgaagcccaccctgtgtgcccatgaaggacgtttccattgtggaacagaagcaagccctaccgagaggagcttcttctgggcagaagttgtgctctttagatatttacgaaagcgcttgtcaagccaaaggctgtgggggcgggcacgtacctaagtctagcgcacctcacgacagagtaccgaccttcctctgcctatccatcccttttcctgtagtgtctcgtgcaatattccagagttcctgctcttctttgcagatgaaaatcttacaccaattttcttccccacgccagggtctgcctgsgagtgatggtgtctcgggaagtcctggagaaccagggagggacgtgagtgtctcttacagctttggagggaggtggcggggcctctgtgctggtatttagcaggtgccctccagatcttccagacactgcctggggcgttgttacccagcaactctttgtttaaagaatttaaagagatttctgaaacctttgtcacccaaatcttgatgcttatggaaaacattcgtccttattgtttgatctgtgccccatctgtgcccgtctcttctcccacccccagtcccgcttactcccctccccaaaactcaccgaacagacactttttaaagtattgtcttcccagctttcaagtatctggccaggttttatcccactaaatgtttaaaaaaatcccaacagaaacacgaaaacgggggcgggggggggggatgagggaatatggggcagggaggctgctggggttgtatatttgtggttgcttttagaattgtttttcgtgtgctgctgtagctcaagcaaggaaacgagactcagttttctagtgaatcgctttttgaaatcgctttcccaaggcatttcagaaatgccctttgtagattagctgattgcatgcctagtctttgagtctttctggaagagctgctaaagccaaagggataaagatcgtctttaggaagccagtggaatgcttccagggcccaggggcaagatggtctggaagctcatacatcctctggggtgcgtcaggatgctgggggcgggtgcccagggcaggtctctgctcagaagctgcctgggactatgcagccttgaacggggccccctcagctgtctccccagtggcagcgacacatttagggatcagcagctggacaatcgggggggtgtatgctgaggtgagcgctctgaaaagaagtaactctcacctgtaatcagatgatatatcatgggccaaagtttgcttttaaaattcagaagaagacttaaaatttgaaaatg

SEQ ID NO: 164 - DNA, 1008 bp, Equus caballus
ggacaaaggggagaccgagggcccatcggcagcatcgggccaaagggtgttcccggagaagacggctaccgagggtaccccggtgatgagggtgggcccggtgatcggggtccaccgggtgtgaacggcactcaaggtttccagggctgccccgggcagagaggaataaagggctctcgtggattcccaggagagaagggtgaattaggagaaatcggacttgatggtcttgacggtgaagatggagacaaaggattgcctgggtcttctggagagaaagggaatcctggaaggaggggtgacaaaggacctaaaggagaccaaggggaaagaggagatgttggaattaggggcgacccgggtgactcagggcgggacagccagcagagaggacccaaaggagaaaccggagacctcgggcccatgggtctgcctgggagtgatggtgtctcgggaagtcctggagaaccagggagggacggtggctttggccgaaggggaccaccaggagctaagggcaacaagggcggtcctggccagcagggcaccgtgggagagcaggggaccagaggtgcacagggtccacctggttccaccggtcctccagggctgatcggcgaacaaggcattcctggacctcggggaagcggaggtgctgtgggcgtccctggagaacgcggccgaaccggtcccttgggaagaaagggcgagcctggagagccgggagcgaagggaggactcgggccccggggcccccgtggggaaacgggagatgacgggcgagacggagttggcagtgaaggacaaaaaggcaaaaaaggagaaagaggattccctggatacccaggtccaaagggtacccgtggtgagccagggacagacggaacactaggacccaaaggcgtcagaggccgaaggggagactcaggacctccaggggcagctggacagaagggagaccctggttacccgggaccatctggtctcaaaggcaacagaggcgactcg

SEQ ID NO: 165 - DNA, 1008 bp, Artificial Sequence
  Description of Artificial Sequence: Synthetic polynucleotide
ggacaaaggggagaccgagggcccatcggcagcatcgggccaaagggtgttcccggagaagacggctaccgagggtaccccggtgatgagggtgggcccggtgatcggggtccaccgggtgtgaacggcactcaaggtttccagggctgccccgggcagagaggaataaagggctctcgtggattcccaggagagaagggtgaattaggagaaatcggacttgatggtcttgacggtgaagatggagacaaaggattgcctgggtcttctggagagaaagggaatcctggaaggaggggtgacaaaggacctaaaggagaccaaggggaaagaggagatgttggaattaggggcgacccgggtgactcagggcgggacagccagcagagaggacccaaaggagaaaccggagacctcgggcccatgggtctgcctgcgagtgatggtgtctcgggaagtcctggagaaccagggagggacggtggctttggccgaaggggaccaccaggagctaagggcaacaagggcggtcctggccagcagggcaccgtgggagagcaggggaccagaggtgcacagggtccacctggttccaccggtcctccagggctgatcggcgaacaaggcattcctggacctcggggaagcggaggtgctgtgggcgtccctggagaacgcggccgaaccggtcccttgggaagaaagggcgagcctggagagccgggagcgaagggaggactcgggccccggggcccccgtggggaaacgggagatgacgggcgagacggagttggcagtgaaggacaaaaaggcaaaaaaggagaaagaggattccctggatacccaggtccaaagggtacccgtggtgagccagggacagacggaacactaggacccaaaggcgtcagaggccgaaggggagactcaggacctccaggggcagctggacagaagggagaccctggttacccgggaccatctggtctcaaaggcaacagaggcgactcg

SEQ ID NO: 166 - DNA, 82 bp, Equus caballus
cccacgccagggtctgccggtctgcctgggagtgatggtgtctcgggaagtcctggagaaccagggagggacgtgagtgtct

SEQ ID NO: 167 - protein, 336 aa, Equus caballus
GQRGDRGPIGSIGPKGVPGEDGYRGYPGDEGGPGDRGPPGVNGTQGFQGCPGQRGIKGSRGFPGEKGELGEIGLDGLDGEDGDKGLPGSSGEKGNPGRRGDKGPKGDQGERGDVGIRGDPGDSGRDSQQRGPKGETGDLGPMGLPGSDGVSGSPGEPGRDGGFGRRGPPGAKGNKGGPGQQGTVGEQGTRGAQGPPGSTGPPGLIGEQGIPGPRGSGGAVGVPGERGRTGPLGRKGEPGEPGAKGGLGPRGPRGETGDDGRDGVGSEGQKGKKGERGFPGYPGPKGTRGEPGTDGTLGPKGVRGRRGDSGPPGAAGQKGDPGYPGPSGLKGNRGDS

SEQ ID NO: 168 - protein, 336 aa, Equus caballus
GQRGDRGPIGSIGPKGVPGEDGYRGYPGDEGGPGDRGPPGVNGTQGFQGCPGQRGIKGSRGFPGEKGELGEIGLDGLDGEDGDKGLPGSSGEKGNPGRRGDKGPKGDQGERGDVGIRGDPGDSGRDSQQRGPKGETGDLGPMGLPASDGVSGSPGEPGRDGGFGRRGPPGAKGNKGGPGQQGTVGEQGTRGAQGPPGSTGPPGLIGEQGIPGPRGSGGAVGVPGERGRTGPLGRKGEPGEPGAKGGLGPRGPRGETGDDGRDGVGSEGQKGKKGERGFPGYPGPKGTRGEPGTDGTLGPKGVRGRRGDSGPPGAAGQKGDPGYPGPSGLKGNRGDS

SEQ ID NO: 169 - DNA, 54 bp, Equus caballus
ggtctgcctgggagtgatggtgtctcgggaagtcctggagaaccagggagggac

SEQ ID NO: 170 - DNA, 54 bp, Artificial Sequence
  Description of Artificial Sequence: Synthetic oligonucleotide
ggtctgcctgcgagtgatggtgtctcgggaagtcctggagaaccagggagggac

SEQ ID NO: 171 - DNA, 20 bp, Artificial Sequence
  Description of Artificial Sequence: Synthetic primer
ttcccagactctcctgtgct

SEQ ID NO: 172 - DNA, 20 bp, Artificial Sequence
  Description of Artificial Sequence: Synthetic primer
agatggggcacagatcaaac

SEQ ID NO: 173 - DNA, 1008 bp, Homo sapiens
gggcagaggggagaccgcgggcccatcggcagcatcgggccaaagggtattcctggagaagacggctaccgaggctatcctggtgatgagggtggacccggtgagcgtggtccgcctggtgtgaacggcactcaaggtttccagggctgcccgggccagagaggagtaaagggctctcggggattcccaggagagaagggcgaagtaggagaaattggactggatggtctggatggtgaagatggagacaaaggattgcctggttcttctggagagaaagggaatcctggaagaaggggtgataaaggacctcgaggagagaaaggagaaagaggagatgttgggattcgaggggacccgggtaacccaggacaagacagccaggagagaggacccaaaggagaaaccggtgacctcggccccatgggtgtcccagggagagatggagtacctggaggacctggagaaactgggaagaatggtggctttggccgaaggggaccccccggagctaagggcaacaagggcggtcctggccagccgggctttgagggagagcaggggaccagaggtgcacagggcccagctggtcctgctggtcctccagggctgataggagaacaaggcatttctggacctcggggaagcggaggtgccgctggtgctcctggagaacgaggcagaaccggtccactgggaagaaagggtgagcccggagagccaggaccaaaaggaggaatcgggaaccggggccctcgtggggagacgggagatgacgggagagacggagttggcagtgaaggacgcagaggcaaaaaaggagaaagaggattccctggatacccaggaccaaagggtaacccaggtgaacctgggctaaatggaacaacaggacccaaaggcatcagaggccgaaggggaaattcgggacctccagggatagttggacagaagggagaccctggctacccaggaccagctggtcccaagggcaacaggggcgactcc

SEQ ID NO: 174 - protein, 336 aa, Homo sapiens
GQRGDRGPIGSIGPKGIPGEDGYRGYPGDEGGPGERGPPGVNGTQGFQGCPGQRGVKGSRGFPGEKGEVGEIGLDGLDGEDGDKGLPGSSGEKGNPGRRGDKGPRGEKGERGDVGIRGDPGNPGQDSQERGPKGETGDLGPMGVPGRDGVPGGPGETGKNGGFGRRGPPGAKGNKGGPGQPGFEGEQGTRGAQGPAGPAGPPGLIGEQGISGPRGSGGAAGAPGERGRTGPLGRKGEPGEPGPKGGIGNRGPRGETGDDGRDGVGSEGRRGKKGERGFPGYPGPKGNPGEPGLNGTTGPKGIRGRRGNSGPPGIVGQKGDPGYPGPAGPKGNRGDS

SEQ ID NO: 175 - protein, 336 aa, Homo sapiens; identical to SEQ ID NO: 174

SEQ ID NO: 176 - protein, 336 aa, Equus caballus; identical to SEQ ID NO: 167

SEQ ID NO: 177 - protein, 59 aa, Unknown
  Description of Unknown: COL6A3 sequence
RGDPGNPGQDSQERGPKGETGDLGPMGVPGRDGVPGGPGETGKNGGFGRRGPPGAKGNK

SEQ ID NO: 178 - protein, 59 aa, Unknown
  Description of Unknown: COL6A3 sequence
RGDPGESGRDSQQRGPKGETGDIGPMGLPGRDGVSGSPGETGKDGGFGRRGPAGAKGNR

SEQ ID NO: 179 - protein, 59 aa, Unknown
  Description of Unknown: COL6A3 sequence
RGDPGDSGRDSQQRGPKGETGDIGPMGLPGRDGVPGRPGDPGKDGGYGRRGPAGAKGNR

SEQ ID NO: 180 - protein, 59 aa, Unknown
  Description of Unknown: COL6A3 sequence
RGDPGDSGRDSQQRGPKGETGDLGPMGLPGSDGVSGSPGEPGRDGGFGRRGPPGAKGNK

SEQ ID NO: 181 - protein, 59 aa, Unknown
  Description of Unknown: COL6A3 sequence
RGDPGDSGQDSQQRGPKGETGDIGPMGLPGRDGVSGSPGEPGKSGGFGRRGPAGAKGNK

SEQ ID NO: 182 - protein, 59 aa, Unknown
  Description of Unknown: COL6A3 sequence
RGDPGDSGRDSQQRGPKGETGDIGPMGLPGRDGVSGRPGETGKDGGFGRRGPAGAKGNK

SEQ ID NO: 183 - protein, 56 aa, Unknown
  Description of Unknown: COL6A3 sequence
RGDPGNSGQDSQQRGAKGETGDIGPVGLPGRDGVSGGPGEPGKSGGFGRRGPAGAK

SEQ ID NO: 184 - protein, 59 aa, Unknown
  Description of Unknown: COL6A3 sequence
RGDPGDSGRDSQQRGPKGETGDIGPMGLPGRDGVSGSPGETGKDGGFGRRGPAGAKGNK

SEQ ID NO: 185 - protein, 59 aa, Papio anubis
RGDPGNPGQDSQQRGPKGETGDLGPMGAPGTDGVPGGPGETGKNGGFGRRGPPGAKGNK

SEQ ID NO: 186 - protein, 59 aa, Macaca mulatta
RGDPGNPGQDSQQRGPKGETGDLGPMGVPGRDGVPGGPGETGKNGGFGRRGPPGAKGNK

SEQ ID NO: 187 - protein, 59 aa, Cebus capucinus imitator
RGDPGNPGQDSQQRGPKGETGDIGPVGVPGRDGVPGGPGETGKNGGFGRRGPPGVKGNK

SEQ ID NO: 188 - protein, 59 aa, Rhinopithecus bieti
RGDPGNPGQDSQQRGPKGEIGDLGPMGVPGRDGVPGGPGETGKNGGFGRRGPPGAKGNK

SEQ ID NO: 189 - protein, 59 aa, Microcebus murinus
RGDPGESGRDSQQRGPKGETGDIGPMGLPGRDGVSGSPGENGRNGGFGRRGPAGAKGNK

SEQ ID NO: 190 - protein, 59 aa, Carlito syrichta
RGDPGDSGRDSQQRGPKGETGDIGPMGLPGRDGVPGRPGETGKNGGFGRRGSAGAKGNK

SEQ ID NO: 191 - protein, 59 aa, Otolemur garnettii
RGDPGESGQDSQQRGPKGETGDIGPMGLPGRDGVSGSPGETGKNGGFGRRGPAGAKGNK

SEQ ID NO: 192 - protein, 59 aa, Propithecus coquereli
RGDPGESGQDSQQRGPKGETGDIGPMGLPGRDGVSGSPGENGKNGGFGRRGPAGAKGNK

SEQ ID NO: 193 - protein, 59 aa, Mus musculus
RGDPGDSGRDSQQRGPKGETGDIGPMGLPGRDGIPGSPGDPGKDGGSGRRGPAGAKGNR

SEQ ID NO: 194 - protein, 59 aa, Rattus norvegicus
RGDPGDSGRDSQQRGPKGETGDIGPMGLPGRDGIPGSPGDPGKDGGFGRRGPAGAKGNR

SEQ ID NO: 195 - protein, 59 aa, Cricetulus griseus
RGDPGDSGRDSQQRGPKGETGDIGPMGLPGRDGIPGRPGDPGKDGGSGRRGPAGAKGNR

SEQ ID NO: 196 - protein, 59 aa, Microtus ochrogaster
RGDPGDSGRDSQQRGPKGETGDIGPMGLPGRDGVPGRPGDPGKDGGFGRRGPAGAKGNR

SEQ ID NO: 197 - protein, 59 aa, Meriones unguiculatus
RGDPGDSGRDSQQRGPKGETGDIGPMGLPGRDGISGRPGDPGKDGGSGRRGPAGAKGNK

SEQ ID NO: 198 - protein, 59 aa, Chinchilla lanigera
RGDPGESGQDSQQRGPKGETGDLGPMGLPGRDGVSGSPGETGKDGGFGRRGPAGAKGNR

SEQ ID NO: 199 - protein, 59 aa, Castor canadensis
RGDPGDSGQDSQQRGPKGETGDIGPMGVPGRDGASGSPGETGKDGGFGRRGPAGVKGNR

SEQ ID NO: 200 - protein, 59 aa, Fukomys damarensis
RGDPGDSGQDNQQRGPKGETGDIGPMGLPGRDGVPGSPGQAGKNGGFGRRGPAGAKGNR

SEQ ID NO: 201 - protein, 59 aa, Pteropus vampyrus
RGVKGDSGRDSQQRGPKGEIGDIGPMGLPGRDGVSGSPGEPGKDGGFGRRGPAGAKGNK

SEQ ID NO: 202 - protein, 59 aa, Manis javanica
RGDPGDSGRDSQQRGPKGETGDLGPMGLPGSDGLPGSSGEPGKNGGFGRRGPAGAKGNR

SEQ ID NO: 203 - protein, 59 aa, Hipposideros armiger
RGDPGEPGRDNQQRGPKGETGDIGPMGLPGRDGAPGRPGEPGESGGFGRRGPAGAKGNK

SEQ ID NO: 204 - protein, 59 aa, Loxodonta africana
RGDPGDSGRDGQQPGPKGETGEIGPMGLPGRDGVSGGPGEPGKDGSFGRRGPAGNKGSK

SEQ ID NO: 205 - protein, 59 aa, Sus scrofa
RGDPGDTGRDSQQRGPKGESGDLGPMGLPGRDGVSGSPGEPGKSGGFGRRGPAGLKGNK

SEQ ID NO: 206 - protein, 59 aa, Balaenoptera acutorostrata scammoni
RGDPGNSGQDSQQRGPKGETGDIGPMGLPGADGVSGGPGEPGKSGGFGRRGPAGAKGNK

SEQ ID NO: 207 - protein, 59 aa, Orcinus orca
RGDPGNSGQDSQQRGPKGETGDIGPMGLPGTDGVSGAPGEPGKSGGFGQRGPAGAKGNK

SEQ ID NO: 208 - protein, 59 aa, Phascolarctos cinereus
RGDPGEIGLDSQQQGAEGEKGEIGPMGMPGLDGTPGGPGVVGKDGGPGRRGPPGVKGNK

SEQ ID NO: 209 - protein, 59 aa, Sarcophilus harrisii
RGDPGEIGKDNQQQGPRGEKGEIGPMGVPGLDGRAGGPGGLGKDGGPGRRGPPGAKGNK

SEQ ID NO: 210 - protein, 59 aa, Ornithorhynchus anatinus
RGDPGDSGLDSRQRGPKGQKGEIGPMGLPGNDGAPGSPGGNGKEGGFGRRGTVGVKGSK

SEQ ID NO: 211 - protein, 59 aa, Unknown
  Description of Unknown: COL6A3 sequence
RGDPGDSGADNTQRGSRGQKGEIGPMGDPGPAGLEGQDGGVGRKGMAGRRGPIGVKGTK

SEQ ID NO: 212 - protein, 59 aa, Haliaeetus leucocephalus
RGDPGDSGADNTQRGSRGQKGEIGPMGEPGPVGLNGQDGGVGRKGMTGRRGPIGVKGTK

SEQ ID NO: 213 - protein, 59 aa, Aquila chrysaetos canadensis
RGDPGDSGADNTQRGSRGQKGEIGPMGEPGPVGLDGQDGGVGRKGMTGRRGPIGVKGTK

SEQ ID NO: 214 - protein, 59 aa, Gallus gallus
RGDPGESGADNTQRGTRGQKGEIGQMGEPGPAGQRGQDGGVGRKGMAGRRGPIGVKGTK

SEQ ID NO: 215 - protein, 59 aa, Picoides pubescens
RGDPGDSGVDNTQRGSRGQKGEIGPMGETGPVGLEGQDGGVGRKGMTGRRGPIGVKGTK

SEQ ID NO: 216 - protein, 59 aa, Meleagris gallopavo
RGDPGDSGADNTQRGTRGQKGEIGQMGEPGPAGQRGPDGGVGRQGMAGRRGPIGVKGTK

SEQ ID NO: 217 - protein, 59 aa, Merops nubicus
RGDPGDSGADNTQRGSKGQKGEIGPMGEPGPVGLNGQDGGVGRKGMTGRRGPIGVKGTK

SEQ ID NO: 218 - protein, 57 aa, Colius striatus
RGDPGDSGADNTQRGSRGQKGEIGPMGEPGPAGLDGQDGGVGRKGMTGRRGPIGVKG

SEQ ID NO: 219 - protein, 59 aa, Apteryx australis mantelli
RGDPGESGADNTQRGSRGQKGEIGPMGEPGGAGANGQNGGIGRKGMAGRRGPIGIKGTK

SEQ ID NO: 220 - protein, 59 aa, Aptenodytes forsteri
RGDPGDSGADNTQRGSRGQKGEIGPMGEPGPAGLDGQDGGVGRKGMTGRRGLIGVKGTK

SEQ ID NO: 221 - protein, 59 aa, Columba livia
RGDPGDSGADNTQRGSRGQKGEIGPMGEPGPAGLEGQEGGVGRRGMAGRRGPIGVKGTK

SEQ ID NO: 222 - protein, 59 aa, Patagioenas fasciata monilis; identical to SEQ ID NO: 221

SEQ ID NO: 223 - protein, 59 aa, Pygoscelis adeliae
RGDPGDSGADNTQRGSRGQKGEIGPMGEPGPVGLDGQGGGVGRKGMTGRRGPIGVKGTK

SEQ ID NO: 224 - protein, 59 aa, Calidris pugnax
RGDPGDSGADNTQRGSRGPKGEIGPMGEPGPAGLDGQDGGVGRKGMPGRRGPIGVKGTK

SEQ ID NO: 225 - protein, 59 aa, Coturnix japonica
RGDPGDSGADNTQRGTRGQKGEIGQMGEPGPAGQRGPDGGVGRQGMAGRRGTIGIKGTK

SEQ ID NO: 226 - protein, 59 aa, Nipponia nippon
RGDPGDSGADNTQRGSRGQKGEIGPMGAPGPVGLGGEEGGVGRKGMTGRRGPIGVKGTK

SEQ ID NO: 227 - protein, 59 aa, Calypte anna
RGDPGDSGADNTQRGSRGQKGEIGPMGEPGPVGVDGQDGGVGRKGMTGRRGPIGPKGTK

SEQ ID NO: 228 - protein, 59 aa, Egretta garzetta
RGDPGDSGADNTQRGSRGQKGEIGPMGEPGPMGLVGQDGGVGRKGMTGRRGQIGVKGTK

SEQ ID NO: 229 - protein, 59 aa, Serinus canaria
RGDPGDSGADNTQRGPRGQKGEIGPMGDPGPAGPEGQDGEVGRRGMAGRRGPIGVKGTK

SEQ ID NO: 230 - protein, 59 aa, Sturnus vulgaris
RGDPGDSGADNTQRGSRGQKGEIGPMGDPGPAGLEGQDGGVGRRGMPGRRGPIGVKGTK

SEQ ID NO: 231 - protein, 59 aa, Taeniopygia guttata
RGDPGDSGADNTQRGPRGQKGEIGPMGDPGPAGLEGPDGEVGRRGMAGRRGPIGVKGTK

SEQ ID NO: 232 - protein, 59 aa, Lonchura striata domestica
RGDPGDSGADNTQRGPRGQKGEIGPMGDPGPAGPEGPDGEVGRRGMAGRRGPIGVKGTK

SEQ ID NO: 233 - protein, 58 aa, Chaetura pelagica
RGDPGDSGADNTQRGPKGQKGEIGPMGEPGPEGVAGQAGGAGRKGMAGRRGPIGVKGT

SEQ ID NO: 234 - protein, 59 aa, Callipepla squamata
RGDPGDSGADNTQRGTRGQKGEIGQMGEPGPVGQRGPDGGVGRMGMAGRRGPIGVKGTK

SEQ ID NO: 235 - protein, 59 aa, Cuculus canorus
RGDPGDSGADNTQRGTRGQKGEIGPMGEPGQAGPEGQEGGVGRKGMTGRRGAIGVKGTK

SEQ ID NO: 236 - protein, 58 aa, Lepidothrix coronata
RGDPGDSGADNTQRGSRGQKGEIGPMGEPGPPGLKGQDGGVGRKGMTGRRGQIGVKGT

SEQ ID NO: 237 - protein, 59 aa, Falco peregrinus
RGDPGDSGADNTQRGSRGPKGEIGPMGEPGLVGLDGQDGGVGRKGMTGRRGQIGIKGTK

SEQ ID NO: 238 - protein, 59 aa, Melopsittacus undulatus
RGDPGDSGADNTQRGPRGQKGEIGQMGEPGPVGPDGQNGEVGRQGMAGRRGPIGVKGTK

SEQ ID NO: 239 - protein, 52 aa, Gekko japonicus
EKGNKGYTGPLGPKGQPGRPGLQGPPGATGRPGVSRPGQRGPQGTPGLKGNK

SEQ ID NO: 240 - protein, 58 aa, Anolis carolinensis
KGQPGRPGVPGIPGPRGEMGLMGPVGNPGLSGVPGNPGIPGIRGSPGFSGLKGRKGSS

SEQ ID NO: 241 - protein, 59 aa, Python bivittatus
RGDPGTAGTDSTQKGPKGQKGELGPAGESGRDGPRGDAGGIGRDGGLGRRGQPGIKGNK

SEQ ID NO: 242 - protein, 59 aa, Protobothrops mucrosquamatus
RGNPGSFGTDSSDRGLKGEKGELGSAGELGRNGPRGDAGGAGRDGALGRRGPPGIKGNK

SEQ ID NO: 243 - protein, 59 aa, Ophiophagus hannah
GKPGTPGFRGERGLMGHGGSPGLPGVSGNPGIPGGRGSPGFPGSKGRKGSFGEKGEPGD

SEQ ID NO: 244 - protein, 59 aa, Thamnophis sirtalis
RGDPGTFGTDSTDRGPKGEKGELGPAGELGRDGPRGDAGEAGRDGSLGKRGPPGIKGNK

SEQ ID NO: 245 - protein, 59 aa, Latimeria chalumnae
RGDPGTPGTNNVRRGPKGQKGEIGPQGDPGNDGTSGTGGPRGKGGSAGRRGPPGTKGEQ

SEQ ID NO: 246 - protein, 59 aa, Rhincodon typus
RGDPGEPGLTNIQKGDKGQRGDMGLVGETGASGRPGSPGASGRRGTQGRRGPPGARGSK

SEQ ID NO: 247 - protein, 59 aa, Callorhinchus milii
RGDPGTSGTDNTQRGIKGQKGDSGIAGDPGTDGTPGQRGPLGKNGATGRRGSAGPRGDK

SEQ ID NO: 248 - protein, 54 aa, Salmo salar
RGDPGTTGQDNNVAGPKGDPGDVGPVGEPGDDGKMGGPGEPGRTGSDGRRGPPG

SEQ ID NO: 249 - protein, 57 aa, Xenopus laevis
RGDPGEPGTNSNNQGPKGLKGNSGRQGETGRDGVQGKRGDNGPNGSQGRRGPPGLKG

SEQ ID NO: 250 - protein, 51 aa, Cyprinus carpio
RGDPGNPGIDNNSRGPKGDIGSPGIQGEPGQDGLSGQIGDEGRPGPNGRRG

SEQ ID NO: 251 - DNA, 529 bp, Equus caballus
ggtccccgagatttctggctttctttgtggcgaggtcgggggaggtgggtgcctgactgttttccccttcctcctgctcatgccccttcctggctttcagatcagggtccaggtgatcgaggggcgccagctgccaggggtgaacatcaagcctgtggtcaaggtcaccgcggccaggcagaccaagcggactcggattcacaggggaaacagcccgctcttcaacgaggtgggagacatggcgttttagggctggtagcttggtgggccttccagattgggagcacccggcagatacctggcaattctttcagtttttgttcatggcgctaactttggtttgagaggtgtgccaggtcctgagtacgttatctgaggaactggagagagggttctagttcttattcctgtcccgggctcctggtgctccacatccctgtcttcctgtggggccagccacccatgctgtcctggagatgacaacctctgagaggtcaggggtggaacaccccagaacttgtcgagtcct

SEQ ID NO: 252 - DNA, 529 bp, Artificial Sequence
  Description of Artificial Sequence: Synthetic polynucleotide
ggtccccgagatttctggctttctttgtggcgaggtcgggggaggtgggtgcctgactgttttccccttcctcctgctcatgccccttcctggctttcagatcagggtccaggtgatcgaggggcgccagctgccaggggtgaacatcaagcctgtggtcaaggtcaccgcggccaggcagaccaagtggactcggattcacaggggaaacagcccgctcttcaacgaggtgggagacatggcgttttagggctggtagcttggtgggccttccagattgggagcacccggcagatacctggcaattctttcagtttttgttcatggcgctaactttggtttgagaggtgtgccaggtcctgagtacgttatctgaggaactggagagagggttctagttcttattcctgtcccgggctcctggtgctccacatccctgtcttcctgtggggccagccacccatgctgtcctggagatgacaacctctgagaggtcaggggtggaacaccccagaacttgtcgagtcct

SEQ ID NO: 253 - DNA, 450 bp, Equus caballus
actggttgcaaactcccaactgtgatcactgacatattccatgagtgtcattttgtggctgaaggtgtgtttgcctggcccggacagaaaggagggtgatggggccttgggtgacaggcactgaccaaagctcttttttctaccccgcagccggccatctaccacattcctggttttgaggtaagtcttgctcttccctcttcttcttcaaactcatggcccgcctctgtgtgtttgcagccccctatgagctaggaagggcagtcaggtgtataccaccaccggcccgccttcagggatggggtgggtgagggccggggtccctggccagctcaggcctttcccgcccttcttccctgagactcagactgtagggacctcatggtcatccagcccacgggctctcagctgggctgcatgttagaatcccttcggcagcttgaaaaatca

SEQ ID NO: 254 - DNA, 450 bp, Artificial Sequence
  Description of Artificial Sequence: Synthetic polynucleotide
actggttgcaaactcccaactgtgatcactgacatattccatgagtgtcattttgtggctgaaggtgtgtttgcctggcccggacagaaaggagggtgatggggccttgggtgacaggcactgaccaaagctcttttttctaccccgcagccggccatctaccacattactggttttgaggtaagtcttgctcttccctcttcttcttcaaactcatggcccgcctctgtgtgtttgcagccccctatgagctaggaagggcagtcaggtgtataccaccaccggcccgccttcagggatggggtgggtgagggccggggtccctggccagctcaggcctttcccgcccttcttccctgagactcagactgtagggacctcatggtcatccagcccacgggctctcagctgggctgcatgttagaatcccttcggcagcttgaaaaatca

SEQ ID NO: 255 - DNA, 499 bp, Equus caballus
ttctttggaactctctccagtgacacttttagctgtaaaattttgtgaacagattttctgctggccattctaaataacacaaaataactatatattgtgtttcctttttatactcactagaataacttctttatcgccttttatatataggttgtattgctgggaaaatacaatgcacagggcttaggttcagatcatgaattaatgctgagatgtaccaaaggacaagaatacgtcaaagtcgtcatgcaaaatgggcgaatgatgggagctgtcttaattggtgaaaccgatttagaagaaacatttgaaaacttgattttaaaccagatgaatctttcagcatatggagaagatctgctggatccagatattgacatagaagattattttgactaaaaaggtcattccaagaaccacataaagttccaaataagacaaaaaagtcacacatcaataaagtaaatgattgcactgatttaatgatgaccacattgaa

SEQ ID NO: 256 - DNA, 499 bp, Artificial Sequence
  Description of Artificial Sequence: Synthetic polynucleotide
ttctttggaactctctccagtgacacttttagctgtaaaattttgtgaacagattttctgctggccattctaaataacacaaaataactatatattgtgtttcctttttatactcactagaataacttctttatcgccttttatatataggttgtattgctgggaaaatacaatgcacagggcttaggttcagatcatgaattaatgctgagatgtaccaaaggacaagaatacgtcaaagtcgtcatgcaaaatgggcgaatgatgggagctgtcttaattggtgaaaccgatttagaagaaacatttgaaaacttgattttaaaccagatgaatctttcagcatatggagaagatctgctgcatccagatattgacatagaagattattttgactaaaaaggtcattccaagaaccacataaagttccaaataagacaaaaaagtcacacatcaataaagtaaatgattgcactgatttaatgatgaccacattgaa

SEQ ID NO: 257 - DNA, 704 bp, Equus caballus
agacctcgggcccatggtacgatgctccttgttcccagactctcctgtgctggaggccagagaaacaaagctcacactggctcgccaggggccgaaggaccatggaagtggtctttgaggctggggagcatatgcggtcaggaacagagggccccgtgaagcccaccctgtgtgcccatgaaggacgtttccattgtggaacagaagcaagccctaccgagaggagcttcttctgggcagaagttgtgctctttagatatttacgaaagcgcttgtcaagccaaaggctgtgggggcgggcacgtacctaagtctagcgcacctcacgacagagtaccgaccttcctctgcctatccatcccttttcctgtagtgtctcgtgcaatattccagagttcctgctcttctttgcagatgaaaatcttacaccaattttcttccccacgccagggtctgcctgggagtgatggtgtctcgggaagtcctggagaaccagggagggacgtgagtgtctcttacagctttggagggaggtggcggggcctctgtgctggtatttagcaggtgccctccagatcttccagacactgcctggggcgttgttacccagcaactctttgtttaaagaatttaaagagatttctgaaacctttgtcacccaaatcttgatgcttatggaaaacattcgtccttattgtttgatc

SEQ ID NO: 258 - DNA, 704 bp, Artificial Sequence
  Description of Artificial Sequence: Synthetic polynucleotide
agacctcgggcccatggtacgatgctccttgttcccagactctcctgtgctggaggccagagaaacaaagctcacactggctcgccaggggccgaaggaccatggaagtggtctttgaggctggggagcatatgcggtcaggaacagagggccccgtgaagcccaccctgtgtgcccatgaaggacgtttccattgtggaacagaagcaagccctaccgagaggagcttcttctgggcagaagttgtgctctttagatatttacgaaagcgcttgtcaagccaaaggctgtgggggcgggcacgtacctaagtctagcgcacctcacgacagagtaccgaccttcctctgcctatccatcccttttcctgtagtgtctcgtgcaatattccagagttcctgctcttctttgcagatgaaaatcttacaccaattttcttccccacgccagggtctgcctgcgagtgatggtgtctcgggaagtcctggagaaccagggagggacgtgagtgtctcttacagctttggagggaggtggcggggcctctgtgctggtatttagcaggtgccctccagatcttccagacactgcctggggcgttgttacccagcaactctttgtttaaagaatttaaagagatttctgaaacctttgtcacccaaatcttgatgcttatggaaaacattcgtccttattgtttgatc

SEQ ID NO: 259 - DNA, 11 bp, Equus caballus
ccaagcggact

SEQ ID NO: 260 - DNA, 11 bp, Artificial Sequence
  Description of Artificial Sequence: Synthetic oligonucleotide
ccaagtggact

SEQ ID NO: 261 - DNA, 11 bp, Artificial Sequence
  Description of Artificial Sequence: Synthetic oligonucleotide
ccaagtggact

SEQ ID NO: 262 - DNA, 11 bp, Equus caballus
accaggaatgt

SEQ ID NO: 263 - DNA, 11 bp, Artificial Sequence
  Description of Artificial Sequence: Synthetic oligonucleotide
accaggaatgt

SEQ ID NO: 264 - DNA, 11 bp, Artificial Sequence
  Description of Artificial Sequence: Synthetic oligonucleotide
accagtaatgt